European Patent Application EP 4 763 998 A1, published June 24, 2026. Title: Small Extracellular Vesicle (sEV) RNA Signature of Head and Neck Squamous Cell Carcinoma (HNSCC) as Biomarker for Tumor Activity, Tumor Stage and HPV Status. Applicant: Universität Ulm. The sequence listing filed with the application follows.

SEQUENCE LISTING (60 sequences)

SEQ ID NO: 1 - RNA, 22 nt, synthetic construct
  source 1..22: mol_type = other RNA
tctacaaaggaaagcgctttct

SEQ ID NO: 2 - RNA, 23 nt, synthetic construct
  source 1..23: mol_type = other RNA
tgattgtagccttttggagtaga

SEQ ID NO: 3 - RNA, 22 nt, synthetic construct
  source 1..22: mol_type = other RNA
caaagcgctcccctttagaggt

SEQ ID NO: 4 - RNA, 19 nt, synthetic construct
  source 1..19: mol_type = other RNA
aatggatttttggagcagg

SEQ ID NO: 5 - RNA, 22 nt, synthetic construct
  source 1..22: mol_type = other RNA
aacacacctattcaaggattca

SEQ ID NO: 6 - RNA, 23 nt, synthetic construct
  source 1..23: mol_type = other RNA
cggggccgtagcactgtctgaga

SEQ ID NO: 7 - RNA, 21 nt, synthetic construct
  source 1..21: mol_type = other RNA
tagtagaccgtatagcgtacg

SEQ ID NO: 8 - RNA, 23 nt, synthetic construct
  source 1..23: mol_type = other RNA
atcagggcttgtggaatgggaag

SEQ ID NO: 9 - RNA, 21 nt, synthetic construct
  source 1..21: mol_type = other RNA
taattttatgtataagctagt

SEQ ID NO: 10 - RNA, 20 nt, synthetic construct
  source 1..20: mol_type = other RNA
aaaagtgattgcagtgtttg

SEQ ID NO: 11 - RNA, 22 nt, synthetic construct
  source 1..22: mol_type = other RNA
aaacaaacatggtgcacttctt

SEQ ID NO: 12 - RNA, 21 nt, synthetic construct
  source 1..21: mol_type = other RNA
atcatagaggaaaatccacgt

SEQ ID NO: 13 - RNA, 20 nt, synthetic construct
  source 1..20: mol_type = other RNA
ctcactgatcaatgaatgca

SEQ ID NO: 14 - RNA, 21 nt, synthetic construct
  source 1..21: mol_type = other RNA
actggacttggtgtcagatgg

SEQ ID NO: 15 - RNA, 23 nt, synthetic construct
  source 1..23: mol_type = other RNA
tgtagtgtttcctactttatgga

SEQ ID NO: 16 - RNA, 22 nt, synthetic construct
  source 1..22: mol_type = other RNA
aaacattcgcggtgcacttctt

SEQ ID NO: 17 - RNA, 23 nt, synthetic construct
  source 1..23: mol_type = other RNA
acttacagacaagagccttgctc

SEQ ID NO: 18 - RNA, 22 nt, synthetic construct
  source 1..22: mol_type = other RNA
tggtttaccgtcccacatacat

SEQ ID NO: 19 - RNA, 22 nt, synthetic construct
  source 1..22: mol_type = other RNA
cttggcacctagcaagcactca

SEQ ID NO: 20 - RNA, 22 nt, synthetic construct
  source 1..22: mol_type = other RNA
taatctcagctggcaactgtga

SEQ ID NO: 21 - RNA, 22 nt, synthetic construct
  source 1..22: mol_type = other RNA
tgtcagtttgtcaaatacccca

SEQ ID NO: 22 - RNA, 22 nt, synthetic construct
  source 1..22: mol_type = other RNA
tatggcactggtagaattcact

SEQ ID NO: 23 - RNA, 22 nt, synthetic construct
  source 1..22: mol_type = other RNA
tagcagcacgtaaatattggcg

SEQ ID NO: 24 - RNA, 21 nt, synthetic construct
  source 1..21: mol_type = other RNA
atcacattgccagggatttcc

SEQ ID NO: 25 - RNA, 23 nt, synthetic construct
  source 1..23: mol_type = other RNA
cctagtaggtgtccagtaagtgt

SEQ ID NO: 26 - RNA, 22 nt, synthetic construct
  source 1..22: mol_type = other RNA
ttttcaactctaatgggagaga

SEQ ID NO: 27 - RNA, 22 nt, synthetic construct
  source 1..22: mol_type = other RNA
tgaggtagtaggttgtatagtt

SEQ ID NO: 28 - RNA, 23 nt, synthetic construct
  source 1..23: mol_type = other RNA
taaatcccatggtgccttctcct

SEQ ID NO: 29 - RNA, 23 nt, synthetic construct
  source 1..23: mol_type = other RNA
tttggcactagcacatttttgct

SEQ ID NO: 30 - RNA, 21 nt, synthetic construct
  source 1..21: mol_type = other RNA
tgcaggaccaagatgagccct

SEQ ID NO: 31 - RNA, 21 nt, synthetic construct
  source 1..21: mol_type = other RNA
tcgtggcctggtctccattat

SEQ ID NO: 32 - RNA, 21 nt, synthetic construct
  source 1..21: mol_type = other RNA
gtgcattgtagttgcattgca

SEQ ID NO: 33 - RNA, 22 nt, synthetic construct
  source 1..22: mol_type = other RNA
gagcttattcataaaagtgcag

SEQ ID NO: 34 - RNA, 23 nt, synthetic construct
  source 1..23: mol_type = other RNA
tgagtgtgtgtgtgtgagtgtgt

SEQ ID NO: 35 - RNA, 4222 nt, synthetic construct
  source 1..4222: mol_type = other RNA
actggagccttagcgggcgcagcagctggaacgggagtactgcgacgcagcccggagtcggccttgtaggggcgaaggtgcagggagatcgcggcgggcgcagtcttgagcgccggagcgcgtccctgcccttagcggggcttgccccagtcgcaggggcacatccagccgctgcggctgacagcagccgcgcgcgcgggagtctgcggggtcgcggcagccgcacctgcgcgggcgaccagcgcaaggtccccgcccggctgggcgggcagcaagggccggggagagggtgcgggtgcaggcgggggccccacagggccaccttcttgcccggcggctgccgctggaaaatgtctcaggagaggcccacgttctaccggcaggagctgaacaagacaatctgggaggtgcccgagcgttaccagaacctgtctccagtgggctctggcgcctatggctctgtgtgtgctgcttttgacacaaaaacggggttacgtgtggcagtgaagaagctctccagaccatttcagtccatcattcatgcgaaaagaacctacagagaactgcggttacttaaacatatgaaacatgaaaatgtgattggtctgttggacgtttttacacctgcaaggtctctggaggaattcaatgatgtgtatctggtgacccatctcatgggggcagatctgaacaacattgtgaaatgtcagaagcttacagatgaccatgttcagttccttatctaccaaattctccgaggtctaaagtatatacattcagctgacataattcacagggacctaaaacctagtaatctagctgtgaatgaagactgtgagctgaagattctggattttggactggctcggcacacagatgatgaaatgacaggctacgtggccactaggtggtacagggctcctgagatcatgctgaactggatgcattacaaccagacagttgatatttggtcagtgggatgcataatggccgagctgttgactggaagaacattgtttcctggtacagaccatattaaccagcttcagcagattatgcgtctgacaggaacaccccccgcttatctcattaacaggatgccaagccatgaggcaagaaactatattcagtctttgactcagatgccgaagatgaactttgcgaatgtatttattggtgccaatcccctggctgtcgacttgctggagaagatgcttgtattggactcagataagagaattacagcggcccaagcccttgcacatgcctactttgctcagtaccacgatcctgatgatgaaccagtggccgatccttatgatcagtcctttgaaagcagggacctccttatagatgagtggaaaagcctgacctatgatgaagtcatcagctttgtgccaccaccccttgaccaagaagagatggagtcctgagcacctggtttctgttctgttgatcccacttcactgtgaggggaaggccttttcacgggaactctccaaatattattcaagtgcctcttgttgcagagatttcctccatggtggaagggggtgtgcgtgcgtgtgcgtgcgtgttagtgtgtgtgcatgtgtgtgtctgtctttgtgggagggtaagacaatatgaacaaactatgatcacagtgactttacaggaggttgtggatgctccagggcagcctccaccttgctcttctttctgagagttggctcaggcagacaagagctgctgtccttttaggaatatgttcaatgcaaagtaaaaaaatatgaattgtccccaatcccggtcatgcttttgccactttggcttctcctgtgaccccaccttgacggtggggcgtagacttgacaacatcccacagtggcacggagagaaggcccataccttctggttgcttcagacctgacaccgtccctcagtgatacgtacagccaaaaaggaccaactggcttctgtgcactagcctgtgattaacttgcttagtatggttctcagatcttgacagtatatttgaaactgtaaatatgtttgtgccttaaaaggagagaagaaagtgtagatagttaaaagactgcagctgctgaagttctgagccgggcaagtcgagagggctgttggacagctgcttgtgggcccggagtaatcaggcagccttcataggcggtcatgtgtgcatgtgagcacatgcgtatatgtgcgtctctctttctccctcacccccaggtgttgccatttctctgcttacccttcacctttggtgcagaggtttcttgaatatctgccccagtagtcagaagcaggttcttgatgtcatgtacttcctgtgtactctttatttctagcagagtgaggatgtgttttgcacgtcttgctatttgagcatgcacagctgcttgtcctgctctcttcaggaggccctggtgtcaggcaggtttgccagtgaagacttcttgggtagtttagatcccatgtcacctcagctgatattatggcaagtgatatcacctctcttcagcccctagtgctattctgtgttgaacacaattgatacttcaggtgcttttgatgtgaaaatcatgaaaagaggaacaggtggatgtatagcatttttattcatgccatctgttttcaaccaactatttttgaggaattatcatgggaaaagaccagggcttttcccaggaatatcccaaacttcggaaacaagttattctcttcactcccaataactaatgctaagaaatgctgaaaatcaaagtaaaaaattaaagcccataaggccagaaactccttttgctgtctttctctaaatatgattactttaaaataaaaaagtaacaaggtgtcttttccactcctatggaaaagggtcttcttggcagcttaacattgacttcttggtttggggagaaataaattttgtttcagaattttgtatattgtaggaatcctttgagaatgtgattccttttgatggggagaaagggcaaattattttaatattttgtattttcaactttataaagataaaatatcctcaggggtggagaagtgtcgttttcataacttgctgaatttcaggcattttgttctacatgaggactcatatatttaagccttttgtgtaataagaaagtataaagtcacttccagtgttggctgtgtgacagaatcttgtatttgggccaaggtgtttccatttctcaatcagtgcagtgatacatgtactccagagggacagggtggaccccctgagtcaactggagcaagaaggaaggaggcagactgatggcgattccctctcacccgggactctccccctttcaaggaaagtgaacctttaaagtaaaggcctcatctcctttattgcagttcaaatcctcaccatccacagcaagatgaattttatcagccatgtttggttgtaaatgctcgtgtgatttcctacagaaatactgctctgaatattttgtaataaaggtctttgcacatgtgaccacatacgtgttaggaggctgcatgctctggaagcctggactctaagctggagctcttggaagagctcttcggtttctgagcataatgctcccatctcctgatttctctgaacagaaaacaaaagagagaatgagggaaattgctattttatttgtattcatgaacttggctgtaatcagttatgccgtataggatgtcagacaataccactggttaaaataaagcctatttttcaaatttagtgagtttctcaagtttattatatttttctcttgtttttatttaatgcacaatatggcattatatcaatatcctttaaactgtgacctggcatacttgtctgacagatcttaatactactcctaacatttagaaaatgttgataaagcttcttagttgtacattttttggtgaagagtatccaggtctttgctgtggatgggtaaagcaaagagcaaatgaacgaagtattaagcattggggcctgtcttatctacactcgagtgtaagagtggccgaaatgacagggctcagcagactgtggcctgagggccaaatctggcccaccacctgtttggtgtagcctgctaagaatggcttttacatttttaaatggttgggaaagaaaaaaaaagaagtagtagattttgtagcatgtgatgtaagtaatgtaaaacttaaattccagtatccataaataaagttttatgagaacaga

SEQ ID NO: 36 - RNA, 3963 nt, synthetic construct
  source 1..3963: mol_type = other RNA
ggggcagccactgcttacactgaagagggaggacgggagaggagtgtgtgtgtgtgtgtgtgtgtgtgtgtgtatgtatgtgtgtgctttatcttatttttctttttggtggtggtggtggaaggggggaggtgctagcagggccagccttgaactcgctggacagagctacagacctatggggcctggaagtgcccgctgagaaagggagaagacagcagaggggttgccgaggcaacctccaagtcccagatcatgtctctgtggggtctggtctccaagatgcccccagaaaaagtgcagcggctctatgtcgactttccccaacacctgcggcatcttctgggtgactggctggagagccagccctgggagttcctggtcggctccgacgccttctgctgcaacttggctagtgccctactttcagacactgtccagcaccttcaggcctcggtgggagagcagggggaggggagcaccatcttgcaacacatcagcacccttgagagcatatatcagagggaccccctgaagctggtggccactttcagacaaatacttcaaggagagaaaaaagctgttatggaacagttccgccacttgccaatgcctttccactggaagcaggaagaactcaagtttaagacaggcttgcggaggctgcagcaccgagtaggggagatccaccttctccgagaagccctgcagaagggggctgaggctggccaagtgtctctgcacagcttgatagaaactcctgctaatgggactgggccaagtgaggccctggccatgctactgcaggagaccactggagagctagaggcagccaaagccctagtgctgaagaggatccagatttggaaacggcagcagcagctggcagggaatggcgcaccgtttgaggagagcctggccccactccaggagaggtgtgaaagcctggtggacatttattcccagctacagcaggaggtaggggcggctggtggggagcttgagcccaagacccgggcatcgctgactggccggctggatgaagtcctgagaaccctcgtcaccagttgcttcctggtggagaagcagcccccccaggtactgaagactcagaccaagttccaggctggagttcgattcctgttgggcttgaggttcctgggggccccagccaagcctccgctggtcagggccgacatggtgacagagaagcaggcgcgggagctgagtgtgcctcagggtcctggggctggagcagaaagcactggagaaatcatcaacaacactgtgcccttggagaacagcattcctgggaactgctgctctgccctgttcaagaacctgcttctcaagaagatcaagcggtgtgagcggaagggcactgagtctgtcacagaggagaagtgcgctgtgctcttctctgccagcttcacacttggccccggcaaactccccatccagctccaggccctgtctctgcccctggtggtcatcgtccatggcaaccaagacaacaatgccaaagccactatcctgtgggacaatgccttctctgagatggaccgcgtgccctttgtggtggctgagcgggtgccctgggagaagatgtgtgaaactctgaacctgaagttcatggctgaggtggggaccaaccgggggctgctcccagagcacttcctcttcctggcccagaagatcttcaatgacaacagcctcagtatggaggccttccagcaccgttctgtgtcctggtcgcagttcaacaaggagatcctgctgggccgtggcttcaccttttggcagtggtttgatggtgtcctggacctcaccaaacgctgtctccggagctactggtctgaccggctgatcattggcttcatcagcaaacagtacgttactagccttcttctcaatgagcccgacggaacctttctcctccgcttcagcgactcagagattgggggcatcaccattgcccatgtcatccggggccaggatggctctccacagatagagaacatccagccattctctgccaaagacctgtccattcgctcactgggggaccgaatccgggatcttgctcagctcaaaaatctctatcccaagaagcccaaggatgaggctttccggagccactacaagcctgaacagatgggtaaggatggcaggggttatgtcccagctaccatcaagatgaccgtggaaagggaccaaccacttcctaccccagagctccagatgcctaccatggtgccttcttatgaccttggaatggcccctgattcctccatgagcatgcagcttggcccagatatggtgccccaggtgtacccaccacactctcactccatccccccgtatcaaggcctctccccagaagaatcagtcaacgtgttgtcagccttccaggagcctcacctgcagatgccccccagcctgggccagatgagcctgccctttgaccagcctcacccccagggcctgctgccgtgccagcctcaggagcatgctgtgtccagccctgaccccctgctctgctcagatgtgaccatggtggaagacagctgcctgagccagccagtgacagcgtttcctcagggcacttggattggtgaagacatattccctcctctgctgcctcccactgaacaggacctcactaagcttctcctggaggggcaaggggagtcggggggagggtccttgggggcacagcccctcctgcagccctcccactatgggcaatctgggatctcaatgtcccacatggacctaagggccaaccccagttggtgatcccagctggagggagaacccaaagagacagctcttctactacccccacagacctgctctggacacttgctcatgccctgccaagcagcagatggggagggtgccctcctatccccacctactcctgggtcaggaggaaaagactaacaggagaatgcacagtgggtggagccaatccactccttcctttctatcattcccctgcccacctccttccagcactgactggaagggaagttcaggctctgagacacaccccaacatgcctgcacctgcagcgcgcacacgcacgcacacacacatacagagctctctgagggtgatggggctgagcaggaggggggctgggtaagagcacaggttagggcatggaaggcttctccgcccattctgacccagggcctaggacggataggcaggaacatacagacacatttacactagaggccagggatagaggatattgggtctcagccctaggggaatgggaagcagctcaagggaccctgggtgggagcataggaggggtctggacatgtggttactagtacaggttttgccctgattaaaaaatctcccaaagccccaaattcctgttagccaggtggaggcttctgatacgtgtatgagactatgcaaaagtacaagggctgagattcttcgtgtatagctgtgtgaacgtgtatgtacctaggatatgttaaatgtatagctggcaccttagttgcatgaccacatagaacatgtgtctatctgcttttgcctacgtgacaacacaaatttgggagggtgagacactgcacagaagacagcagcaagtgtgctggcctctctgacatatgctaacccccaaatactctgaatttggagtctgactgtgcccaagtgggtccaagtggctgtgacatctacgtatggctccacacctccaatgctgcctgggagccagggtgagagtctgggtccaggcctggccatgtggccctccagtgtatgagagggccctgcctgctgcatcttttctgttgccccatccaccgccagcttcccttcactcccctatcccattctccctctcaaggcaggggtcatagatcctaagccataaaataaattttattccaaaataacaaaataaataatctactgtacacaatctgaaaa

SEQ ID NO: 37 - RNA, 3991 nt, synthetic construct
  source 1..3991: mol_type = other RNA
agccaattctgaccgtgtcaacgaatcatccacgcacctgcagctctgctgagagagtgcaagccgtgggaattcagcagctgaatatcaagacctttgaattcaacaagaagttaagacatttatagttgtctaacaacagactgaagattgtggcttggtattcactggcaggtttcagacatttagatctttcttttaatgactaacaccatgcctatctgtggagaagctggcaacatgtcacacctggaaattgtttttcaacattaatactattatttggcagtaatccagattgcttttgccaccaacctgaagacatatagaggcagaaggacaggaataattctatttgtttcctgttttgaaacttccatctgtaaggctatcaaaaggagatgtgagagagggtattgagtctggcctgacaatgcagttcttaaaccaaaggtccattatgcttctcctctctgagaatcctgacttacctcaacaacggagacatggcacagtagccagcttggagacttctcagccaatgctctgagatcaagtcgaagacccaatatacagggttttgagctcatcttcatcattcatatgaggaaataagtggtaaaatccttggaaatacaatgagactcatcagaaacatttacatattttgtagtattgttatgacagcagagggtgatgctccagagctgccagaagaaagggaactgatgaccaactgctccaacatgtctctaagaaaggttcccgcagacttgaccccagccacaacgacactggatttatcctataacctcctttttcaactccagagttcagattttcattctgtctccaaactgagagttttgattctatgccataacagaattcaacagctggatctcaaaacctttgaattcaacaaggagttaagatatttagatttgtctaataacagactgaagagtgtaacttggtatttactggcaggtctcaggtatttagatctttcttttaatgactttgacaccatgcctatctgtgaggaagctggcaacatgtcacacctggaaatcctaggtttgagtggggcaaaaatacaaaaatcagatttccagaaaattgctcatctgcatctaaatactgtcttcttaggattcagaactcttcctcattatgaagaaggtagcctgcccatcttaaacacaacaaaactgcacattgttttaccaatggacacaaatttctgggttcttttgcgtgatggaatcaagacttcaaaaatattagaaatgacaaatatagatggcaaaagccaatttgtaagttatgaaatgcaacgaaatcttagtttagaaaatgctaagacatcggttctattgcttaataaagttgatttactctgggacgaccttttccttatcttacaatttgtttggcatacatcagtggaacactttcagatccgaaatgtgacttttggtggtaaggcttatcttgaccacaattcatttgactactcaaatactgtaatgagaactataaaattggagcatgtacatttcagagtgttttacattcaacaggataaaatctatttgcttttgaccaaaatggacatagaaaacctgacaatatcaaatgcacaaatgccacacatgcttttcccgaattatcctacgaaattccaatatttaaattttgccaataatatcttaacagacgagttgtttaaaagaactatccaactgcctcacttgaaaactctcattttgaatggcaataaactggagacactttctttagtaagttgctttgctaacaacacacccttggaacacttggatctgagtcaaaatctattacaacataaaaatgatgaaaattgctcatggccagaaactgtggtcaatatgaatctgtcatacaataaattgtctgattctgtcttcaggtgcttgcccaaaagtattcaaatacttgacctaaataataaccaaatccaaactgtacctaaagagactattcatctgatggccttacgagaactaaatattgcatttaattttctaactgatctccctggatgcagtcatttcagtagactttcagttctgaacattgaaatgaacttcattctcagcccatctctggattttgttcagagctgccaggaagttaaaactctaaatgcgggaagaaatccattccggtgtacctgtgaattaaaaaatttcattcagcttgaaacatattcagaggtcatgatggttggatggtcagattcatacacctgtgaataccctttaaacctaaggggaactaggttaaaagacgttcatctccacgaattatcttgcaacacagctctgttgattgtcaccattgtggttattatgctagttctggggttggctgtggccttctgctgtctccactttgatctgccctggtatctcaggatgctaggtcaatgcacacaaacatggcacagggttaggaaaacaacccaagaacaactcaagagaaatgtccgattccacgcatttatttcatacagtgaacatgattctctgtgggtgaagaatgaattgatccccaatctagagaaggaagatggttctatcttgatttgcctttatgaaagctactttgaccctggcaaaagcattagtgaaaatattgtaagcttcattgagaaaagctataagtccatctttgttttgtctcccaactttgtccagaatgagtggtgccattatgaattctactttgcccaccacaatctcttccatgaaaattctgatcatataattcttatcttactggaacccattccattctattgcattcccaccaggtatcataaactgaaagctctcctggaaaaaaaagcatacttggaatggcccaaggataggcgtaaatgtgggcttttctgggcaaaccttcgagctgctattaatgttaatgtattagccaccagagaaatgtatgaactgcagacattcacagagttaaatgaagagtctcgaggttctacaatctctctgatgagaacagattgtctataaaatcccacagtccttgggaagttggggaccacatacactgttgggatgtacattgatacaacctttatgatggcaatttgacaatatttattaaaataaaaaatggttattcccttcatatcagtttctagaaggatttctaagaatgtatcctatagaaacaccttcacaagtttataagggcttatggaaaaaggtgttcatcccaggattgtttataatcatgaaaaatgtggccaggtgcagtggctcactcttgtaatcccagcactatgggaggccaaggtgggtgacccacgaggtcaagagatggagaccatcctggccaacatggtgaaaccctgtctctactaaaaatacaaaaattagctgggcgtgatggtgcacgcctgtagtcccagctacttgggaggctgaggcaggagaatcgcttgaacccgggaggtggcagttgcagtgagctgagatcgagccactgcactccagcctggtgacagagcgagactccatctcaaaaaaaagaaaaaaaaaaaagaaaaaaatggaaaacatcctcatggccacaaaataaggtctaattcaataaattatagtacattaatgtaatataatattacatgccactaaaaagaataaggtagctgtatatttcctggtatggaaaaaacatattaatatgttataaactattaggttggtgcaaaactaattgtggtttttgccattgaaatggcattgaaataaaagtgtaaagaaatctataccagatgtagtaacagtggtttgggtctgggaggttggattacagggagcatttgatttctatgttgtgtatttctataatgtttgaattgtttagaatgaatctgtatttcttttataagtagaaaaaaaataaagatagtttttacagccta

SEQ ID NO: 38 - RNA, 934 nt, synthetic construct
  source 1..934: mol_type = other RNA
agttacacgttttcctccaaggagcctcggacgttgtcacgggtttggggtcggggacagagcggtgaccatggccaggctggcgttgtctcctgtgcccagccactggatggtggcgttgctgctgctgctctcagctgagccagtaccagcagccagatcggaggaccggtaccggaatcccaaaggattcagcaccttggcacagctgaagcagaggaacacgctgaaggatggtatcatcatgatccagacgctgctgatcatcctcttcatcatcgtgcctatcttcctgctgctggacaaggatgacagcaaggctggcatggaggaagatcacacctacgagggcctggacattgaccagacagccacctatgaggacatagtgacgctgcggacaggggaagtgaagtggtctgtaggtgagcacccaggccaggagtgagagccaggtcgccccatgacctgggtgcaggctccctggcctcagtgactgcttcggagctgcctggctcatggcccaacccctttcctggaccccccagctggcctctgaagctggcccaccagagctgccatttgtctccagcccctggtccccagctcttgccaaagggcctggagtagaaggacaacagggcagcaacttggagggagttctctggggatggacgggacccagccttctgggggtgctatgaggtgatccgtccccacacatgggatgggggaggcagagactggtccagagcccgcaaatggactcggagccgagggcctcccagcagagcttgggaagggccatggacccaactgggccccagaagagccacaggaacatcattcctctcccgcaaccactcccaccccagggaggccctggcctccagtgccttcccccgtggaataaacggtgtgtcctgagaaacca

SEQ ID NO: 39 - RNA, 408 nt, synthetic construct
  source 1..408: mol_type = other RNA
atgtctcttgtcagctgtctttcagaagacctggtggggcaagtccgtgggcatcatgttgaccgagctggagaaagccttgaactctatcatcgacgtctaccacaagtactccctgataaaggggaatttccatgccgtctacagggatgacctgaagaaattgctagagaccgagtgtcctcagtatatcaggaaaaagggtgcagacgtctggttcaaagagttggatatcaacactgatggtgcagttaacttccaggagttcctcattctggtgataaagatgggcgtggcagcccacaaaaaaagccatgaagaaagccacaaagagtagctgagttactgggcccagaggctgggcccctggacatgtacctgcagaataataaagtcatcaatacctca

SEQ ID NO: 40 - RNA, 1708 nt, synthetic construct
  source 1..1708: mol_type = other RNA
gctcttgtcgatttcctgtagtgaatcaggcaccggagtgcaggttcgggggtggaatccttgggccgctgggcaagcggcgagacctggccagggccagcgagccgaggacagagggcgcacggagggccgggccgcagccccggccgcttgcagaccccgccatggacccgttcctggtgctgctgcactcggtgtcgtccagcctgtcgagcagcgagctgaccgagctcaagttcctatgcctcgggcgcgtgggcaagcgcaagctggagcgcgtgcagagcggcctagacctcttctccatgctgctggagcagaacgacctggagcccgggcacaccgagctcctgcgcgagctgctcgcctccctgcggcgccacgacctgctgcggcgcgtcgacgacttcgaggcgggggcggcggccggggccgcgcctggggaagaagacctgtgtgcagcatttaacgtcatatgtgataatgtggggaaagattggagaaggctggctcgtcagctcaaagtctcagacaccaagatcgacagcatcgaggacagatacccccgcaacctgacagagcgtgtgcgggagtcactgagaatctggaagaacacagagaaggagaacgcaacagtggcccacctggtgggggctctcaggtcctgccagatgaacctggtggctgacctggtacaagaggttcagcaggcccgtgacctccagaacaggagtggggccatgtccccgatgtcatggaactcagacgcatctacctccgaagcgtcctgatgggccgctgctttgcgctggtggaccacaggcatctacacagcctggactttggttctctccaggaaggtagcccagcactgtgaagacccagcaggaagccaggctgagtgagccacagaccacctgcttctgaactcaagctgcgtttattaatgcctctcccgcaccaggccgggcttgggccctgcacagatatttccatttcttcctcactatgacactgagcaagatcttgtctccactaaatgagctcctgcgggagtagttggaaagttggaaccgtgtccagcacagaaggaatctgtgcagatgagcagtcacactgttactccacagcggaggagaccagctcagaggcccaggaatcggagcgaagcagagaggtggagaactgggatttgaacccccgccatccttcaccagagcccatgctcaaccactgtggcgttctgctgcccctgcagttggcagaaaggatgttttgtcccatttccttggaggccaccgggacagacctggacactagggtcaggcggggtgctgtggtggggagaggcatggctggggtgggggtggggagacctggttggccgtggtccagctcttggcccctgtgtgagttgagtctcctctctgagactgctaagtaggggcagtgatggttgccaggacgaattgagataatatctgtgaggtgctgatgagtgattgacacacagcactctctaaatcttccttgtgaggattatgggtcctgcaattctacagtttcttactgttttgtatcaaaatcactatctttctgataacagaattgccaaggcagcgggatctcgtatctttaaaaagcagtcctcttattcctaaggtaatcctattaaaacacagctttacaacttccatactacaaaaaa

SEQ ID NO: 41 - RNA, 2201 nt, synthetic construct
  source 1..2201: mol_type = other RNA
gcccgctcgcccgcgcgccccaggacccaaagccgggctccaagtcggcgccccacgtcgaggctccgccgcagcctccggagttggccgcagacaagaaggggagggagcgggagagggaggagagctccgaagcgagagggccgagcgccatgcgccgcgccagcagagactacaccaagtacctgcgtggctcggaggagatgggcggcggccccggagccccgcacgagggccccctgcacgccccgccgccgcctgcgccgcaccagccccctgccgcctcccgctccatgttcgtggccctcctggggctggggctgggccaggttgtctgcagcgtcgccctgttcttctatttcagagcgcagatggatcctaatagaatatcagaagatggcactcactgcatttatagaattttgagactccatgaaaatgcagattttcaagacacaactctggagagtcaagatacaaaattaatacctgattcatgtaggagaattaaacaggcctttcaaggagctgtgcaaaaggaattacaacatatcgttggatcacagcacatcagagcagagaaagcgatggtggatggctcatggttagatctggccaagaggagcaagcttgaagctcagccttttgctcatctcactattaatgccaccgacatcccatctggttcccataaagtgagtctgtcctcttggtaccatgatcggggttgggccaagatctccaacatgacttttagcaatggaaaactaatagttaatcaggatggcttttattacctgtatgccaacatttgctttcgacatcatgaaacttcaggagacctagctacagagtatcttcaactaatggtgtacgtcactaaaaccagcatcaaaatcccaagttctcataccctgatgaaaggaggaagcaccaagtattggtcagggaattctgaattccatttttattccataaacgttggtggattttttaagttacggtctggagaggaaatcagcatcgaggtctccaacccctccttactggatccggatcaggatgcaacatactttggggcttttaaagttcgagatatagattgagccccagtttttggagtgttatgtatttcctggatgtttggaaacattttttaaaacaagccaagaaagatgtatataggtgtgtgagactactaagaggcatggccccaacggtacacgactcagtatccatgctcttgaccttgtagagaacacgcgtatttacagccagtgggagatgttagactcatggtgtgttacacaatggtttttaaattttgtaatgaattcctagaattaaaccagattggagcaattacggggtgaccttatgagaaactgcatgtgggctatgggaggggttggtccctggtcatgtgccccttcgcagctgaagtggagagggtgtcatctagcgcaattgaaggatcatctgaaggggcaaattcttttgaattgttacatcatgctggaacctgcaaaaaatactttttctaatgaggagagaaaatatatgtatttttatataatatctaaagttatatttcagatgtaatgttttctttgcaaagtattgtaaattatatttgtgctatagtatttgattcaaaatatttaaaaatgtcttgctgttgacatatttaatgttttaaatgtacagacatatttaactggtgcactttgtaaattccctggggaaaacttgcagctaaggaggggaaaaaaatgttgtttcctaatatcaaatgcagtatatttcttcgttctttttaagttaatagattttttcagacttgtcaagcctgtgcaaaaaaattaaaatggatgccttgaataataagcaggatgttggccaccaggtgcctttcaaatttagaaactaattgactttagaaagctgacattgccaaaaaggatacataatgggccactgaaatctgtcaagagtagttatataattgttgaacaggtgtttttccacaagtgccgcaaattgtaccttttttgttttttcaaaatagaaaagttattagtggtttatcagcaaaaaagtccaattttaatttagtaaatgttatcttatactgtacaataaaaacattgcctttgaatgttaattttttggtacaaaaataaatttatatgaaaacctgc

SEQ ID NO: 42 - RNA, 8677 nt, synthetic construct
  source 1..8677: mol_type = other RNA
aggtagcaggtttggctgcgcgggggccgcgcgtcggagtttccccctttctagggtgaggatggttctacacagccacccggagttccttagttgaaaggtgcgccctgctgtgacagaatgtggtaattgtaatctttaacattttcatgtaaaacatatttcctgatcatctttccattgtcttcatggaaaattgataaatatttgtgccttccaactctcgtcttggttgaatgacttcatcttaatacaacatggacaccacgttgctgaaaacatgctttgggactgccactgaatttatcttttgcggttttatgacaaagttattagtagtttcccttttttgaattagtattttgaagttaatatcacaatgagttcaggcttatggagccaagaaaaagtcacttcaccctactgggaagagcggattttttacttgcttcttcaagaatgcagcgttacagacaaacaaacacaaaagctccttaaagtaccgaagggaagtataggacagtatattcaagatcgttctgtggggcattcaaggattccttctgcaaaaggcaagaaaaatcagattggattaaaaattctagagcaacctcatgcagttctctttgttgatgaaaaggatgttgtagagataaatgaaaagttcacagagttacttttggcaattaccaattgtgaggagaggttcagcctgtttaaaaacagaaacagactaagtaaaggcctccaaatagacgtgggctgtcctgtgaaagtacagctgagatctggggaagaaaaatttcctggagttgtacgcttcagaggacccctgttagcagagaggacagtctccggaatattctttggagttgaattgctggaagaaggtcgtggtcaaggtttcactgacggggtgtaccaagggaaacagctttttcagtgtgatgaagattgtggcgtgtttgttgcattggacaagctagaactcatagaagatgatgacactgcattggaaagtgattacgcaggtcctggggacacaatgcaggtcgaacttcctcctttggaaataaactccagagtttctttgaaggttggagaaacaatagaatctggaacagttatattctgtgatgttttgccaggaaaagaaagcttaggatattttgttggtgtggacatggataaccctattggcaactgggatggaagatttgatggagtgcagctttgtagttttgcgtgtgttgaaagtacaattctattgcacatcaatgatatcatcccagctttatcagagagtgtgacgcaggaaaggaggcctcccaaacttgcctttatgtcaagaggtgttggggacaaaggttcatccagtcataataaaccaaaggctacaggatctacctcagaccctggaaatagaaacagatctgaattattttataccttaaatgggtcttctgttgactcacaaccacaatccaaatcaaaaaatacatggtacattgatgaagttgcagaagaccctgcaaaatctcttacagagatatctacagactttgaccgttcttcaccaccactccagcctcctcctgtgaactcactgaccaccgagaacagattccactctttaccattcagtctcaccaagatgcccaataccaatggaagtattggccacagtccactttctctgtcagcccagtctgtaatggaagagctaaacactgcacccgtccaagagagtccacccttggccatgcctcctgggaactcacatggtctagaagtgggctcattggctgaagttaaggagaaccctcctttctatggggtaatccgttggatcggtcagccaccaggactgaatgaagtgctcgctggactggaactggaagatgagtgtgcaggctgtacggatggaaccttcagaggcactcggtatttcacctgtgccctgaagaaggcgctgtttgtgaaactgaagagctgcaggcctgactctaggtttgcatcattgcagccggtttccaatcagattgagcgctgtaactctttagcatttggaggctacttaagtgaagtagtagaagaaaatactccaccaaaaatggaaaaagaaggcttggagataatgattgggaagaagaaaggcatccagggtcattacaattcttgttacttagactcaaccttattctgcttatttgcttttagttctgttctggacactgtgttacttagacccaaagaaaagaacgatgtagaatattatagtgaaacccaagagctactgaggacagaaattgttaatcctctgagaatatatggatatgtgtgtgccacaaaaattatgaaactgaggaaaatacttgaaaaggtggaggctgcatcaggatttacctctgaagaaaaagatcctgaggaattcttgaatattctgtttcatcatattttaagggtagaacctttgctaaaaataagatcagcaggtcaaaaggtacaagattgttacttctatcaaatttttatggaaaaaaatgagaaagttggcgttcccacaattcagcagttgttagaatggtcttttatcaacagtaacctgaaatttgcagaggcaccatcatgtctgattattcagatgcctcgatttggaaaagactttaaactatttaaaaaaatttttccttctctggaattaaatataacagatttacttgaagacactcccagacagtgccggatatgtggagggcttgcaatgtatgagtgtagagaatgctacgacgatccggacatctcagctggaaaaatcaagcagttttgtaaaacctgcaacactcaagtccaccttcatccgaagaggctgaatcataaatataacccagtgtcacttcccaaagacttacccgactgggactggagacacggctgcatcccttgccagaatatggagttatttgctgttctctgcatagaaacaagccactatgttgcttttgtgaagtatgggaaggacgattctgcctggctcttctttgacagcatggccgatcgggatggtggtcagaatggcttcaacattcctcaagtcaccccatgcccagaagtaggagagtacttgaagatgtctctggaagacctgcattccttggactccaggagaatccaaggctgtgcacgaagactgctttgtgatgcatatatgtgcatgtaccagagtccaacaatgagtttgtacaaataactggggtcatcgggaaaggcaaagaaactgaaggcagagtcctaacgttgcatcttattcgagctggcagttctgttcacgtccattgccggcaatggatgtctttgtggtgatgatccttcagaaaaggatgcctctgtttaaaaacaaattgcttttgtgtccctgaagtatttaataagaagcattttgcactctagaaagtatgtttgtgttggttttttaagaagtctaaatgaagttattaatacctgaagctttaagttaagtgcattgatcatatgatatttttggaagcatacaattttaattgtggaagtttaaagcctcttttagtccattgagaatgtaaataaatgtgtcttctttatggaccaaggatatgaaatcatttttcttttgtagctaacggttgccttgaggaagaaataatttggttttattaagagtctactctcaatccagttattagagatgtactgagtttgatttgttaatcctttctatatactgctgatcttgcatgtctacaatctgctcagtttttctgtgtttctgcaatagtggtcagaaaaatacttaaattcccttaatggtgttgttttctatttgttctggttttgagataaatgagtgattctgtccccaaatgtccatttttgaagtgattttcctggaggattagggtatttagcagttgaagctcttcattcatagtagttactgtcagctaacaggttttttaaggcttttaactattaatattttatggaatggggcaaagtaaattgatgaaagaattggagtgataatagtcctttacaaacatacagtccataagaaaatgaatttggcatatagaattattacaatttcctgggagagatggatatttaaacctctattattttagacaagactgtctagaacttaagtttgatctgtcagccagtactcccattaaattcagtgtagtttcacttgatagaatcagatatgttatcgaaatgttagcagcagcttcatcctccttctgattaaagtaagtagaaatgggatgttttgtttaataacagccatagtgtgtgtttagaccacagcggatgttgtagaccaggaccatagatgatacatgtcagtgctgtggaatgtgcattctctgagtgttgttttgtggtatcattgtctttcctgaatgactttctaactgtgcagaaaggcagaaaagtcatcatatgtatatgtcatatgactttataaaatatttaatgtgacaaaaagtggaaagaatctttacaaaccctgcaattacttttttaaaggcacttttactctttggttttatcattccattttgctaatatttactagctttataaattacagtaaggtacaaaaactcatcttgtaatattttcatttttgaagtgaaaaagtacatatattttgcacaaggttttatactgctaagtgcttggttggggtggtgagatgatgattagatcaggggtgaggctgagagactctgggtttagggctagccctgcctccatctcccttgggtaaaatgaagggtgtggggtaaaagatgcataaggccttttctagctctgacagcctagaagtccaatcaccctgtaataaatatgtgttgaatgaagaaatgggtgaatgagcttgtcaatgtgattttaaaaaattgactacctggaggaatgattaggaatctaaatgaagccagccctcggtatctgcaggtttctcatccatggattcaaccaactgcaaatggaaaatacgattttttttaaaaaaaggatggttacatccgtattgaacatgtacagacttttttcttgtcattattctctgaacaatacaagaactctttatgtagcatttacatttattaggtattataagtaatctagagattatttaattaaaatatacaggaggatgtgtgtcagttatatgcaaattctgtaccattttgtatcagggaattgagcatcttcagatgttggtatctgcagggatcctggaaccaaacccctgcagatactaagggctgacgatctaggtaagactggatttaacagttggaaaaaaaaaaaaaaaaggagagagaagacagttcctttcctgtagaaattaaaacaaaatacaaattgaggaagctctgctacccaggctgtcatggtagagaacttgaagaagacctgtttggatggacacctggtttcaaaagtcaggtgtggagactgttaaatgggagggcctcatccataaatgatttctggcaacgtcttcttcaggtggagcttgacgtctttttaatgttacttggggagggagtgctcattaagggatgccagggccagctctggtggttcctggggaggctgcgtccttccctgcttctgcatgtcatgaggcagcaggaaggtttcccctgcacctgtctgtcctggctccctctgggtagccccctactgttctgtgcttcagcacagcctggtttgtcaagaggcacatagttggggctgggctgcatggcacaggggcttatgtgcctgctggttatttaattttcagccttaagttttctttaatattttcctgttggctatttaaaggttttggttatcttttattccttatctacaatcaagatgacaatgtaattgaattatcttatttataacacggttcgtgattcatgattcatgattacaagtagaaaatatgtcatgttcctcacctccaaataaatatgtgtgtgtctgtgtgtgtgtatatatgtatgtggcggagagggagagagtggggaaggagagcagtgttatcatacatagagaggctaaatgtgtcccatccctcactgtcagctttataaaggagtttgactccatccacagaagaatgttttataagactaggaaaacacgttgaaaactaggataaacagcaacaaaaatcaactaaatatgttgttactgttgctaaggattttctccttagaataatttaggatttttaaaaatttctgtttgccaaatgctgtagataaatggccagattcttcctatccctaggattcctttattattttttttcacagattttgagaacaagggggagagatagtatggaagattaagattccattaatcttatagaactgtgttgtcacccaaattcctgcttgtttgaacatggcatcttcatagattcaggattcactaccctctatagctggatcttgaaaattatctggccagataattttgcatctgcttggatgattgtagactgagatgtgagtggaggataaagtattagacttttgctgagtaactgccaaccaagaagtatttatcggacacttactaggtgcctaggattgtatcagagggaatatgaaatgtgtccctgccctacctagttttaacgacagaatatctattaaaggctacttagctgaagggtaagggtgacaggtctaggggaagctttgggaggtggtgtgctgtgacagaaaaagtggcagagtagggacgagagacctgcattctagccctgtttctgtcacttgctctgtacacttagacaacagcttgacctcttgagctttagtttcctcctctgcataatgagagggttagactactgaattgtatgggaaaaaaatacaaattcctgggtcctaggccatgcctgctgaatccgactgttcaggaagaggcctaggaaatctgtgagggaatccccaggggaatctcgtgaccagccaggtgtgaaatctgctaactggaagatctcaaagcttccttcactttttgtgattttgtggtcatgtaacgttactgtattattctacgtaaatgtgggtacttggatgtttatcatactgtttctctgtgtttacatactaatttgtgtaagaaatgcattttagtctgtgtacctcaacctgctgtttgtttcctagaggtgttagtagtctttaaatacaagtaagacttaagaggatatttgatgttatttacctggatattttcttccccttttatttatttagaggaaattgagattctaggagccaaaaaaatgaaaacaaaattctaaggcaaagttaaagaaaaaaattacattatttcttaccatttgctactttataatgaaaatttaaaaattatatgggaagatttttctctgggataacaaatccttgtcataaagtaagaggtctttttaaagtaggtaggctataaggcctgtaatttaaaataatactcctttctctagggtttggtgcaattctccattaatgaagataacatttgaattccccaaagcaggtgaggagtcggggaggagaaagcgatgttaaaatgaaaactcactgcaaaagaggaggcagaggaagaaggaatgtaaaccccttaaagcagatgtgtgtggggccttatgaagaccaggattctgcgggtgtcaggggattgcccctcttgacagagactagggttttagactgaggcttcctgcagggtgttcgcattgcccttctccgttccccttcagacctttctggggagaagaggtgggaggaggggagaaagactgttcatcttattctgaatcctggagcagctgaaggttttctcttgagtcaggatgcagtggtaatgcattaaccagcaagtgtggccaaggataatgaaaaagtgggaaaggaaggtcctcctcctccctgattgtagcatccagcagtctctgtagccaggttactcaagaaccacatttgatttcctggccctttgccttggcagtgatggcatttttatttcactgtgttttaaagtcttcatttatttttataacatgggttagggagaagggccacaaatggagggattgtcctttcaagcaccacagcttcagataaaattagtactttcaaatattgtccactttaacttaaaaaattctagagggattatattggagactcaactgcccttggttttagtttataaaatggcctagtactgtggaattttaattttagaaagtcttagcatcagatcataaacattcattaaaagaactcacatcccatctgaaacttcccaggggagttgggattcttagtagattggtagaaaggggctcattttctactgcatttcccatttttggtatcttgttcagcatgttttatttttatttcttgtctgcagaacatcctatatttatgagaacattctttaagaagaccaccacatagaataccccttcctatcagctcgctctgatttagccttaattttgttaaattttttagagatgaatgaagtgctgctgtggaaagaaatgtacatatactatttctgtatcattaaaattacatttttatggttc

SEQ ID NO: 43 - RNA, 5129 nt, synthetic construct
  source 1..5129: mol_type = other RNA
atcattttcctctttcaccctgtctaggttgccagcaaatcccacgggcctcctgacgctgcccctggggccacaggtccctcgagtgctggaaggatgaaggattcctgcatcactgtgatggccatggcgctgctgtctgggttctttttcttcgcgccggcctcgagctacaacctggacgtgcggggcgcgcggagcttctccccaccgcgcgccgggaggcactttggataccgcgtcctgcaggtcggaaacggggtcatcgtgggagctccaggggaggggaacagcacaggaagcctctatcagtgccagtcgggcacaggacactgcctgccagtcaccctgagaggttccaactatacctccaagtacttgggaatgaccttggcaacagaccccacagatggaagcattttggcctgtgaccctgggctgtctcgaacgtgtgaccagaacacctatctgagtggcctgtgttacctcttccgccagaatctgcagggtcccatgctgcaggggcgccctggttttcaggaatgtatcaagggcaacgtagacctggtatttctgtttgatggttcgatgagcttgcagccagatgaatttcagaaaattctggacttcatgaaggatgtgatgaagaaactcagcaacacttcgtaccagtttgctgctgttcagttttccacaagctacaaaacagaatttgatttctcagattatgttaaacggaaggaccctgatgctctgctgaagcatgtaaagcacatgttgctgttgaccaatacctttggtgccatcaattatgtcgcgacagaggtgttccgggaggagctgggggcccggccagatgccaccaaagtgcttatcatcatcacggatggggaggccactgacagtggcaacatcgatgcggccaaagacatcatccgctacatcatcgggattggaaagcattttcagaccaaggagagtcaggagaccctccacaaatttgcatcaaaacccgcgagcgagtttgtgaaaattctggacacatttgagaagctgaaagatctattcactgagctgcagaagaagatctatgtcattgagggcacaagcaaacaggacctgacttccttcaacatggagctgtcctccagcggcatcagtgctgacctcagcaggggccatgcagtcgtgggggcagtaggagccaaggactgggctgggggctttcttgacctgaaggcagacctgcaggatgacacatttattgggaatgaaccattgacaccagaagtgagagcaggctatttgggttacaccgtgacctggctgccctcccggcaaaagacttcgttgctggcctcgggagcccctcgataccagcacatgggccgagtgctgctgttccaagagccacagggcggaggacactggagccaggtccagacaatccatgggacccagattggctcttatttcggtggggagctgtgtggcgtcgacgtggaccaagatggggagacagagctgctgctgattggtgccccactgttctatggggagcagagaggaggccgggtgtttatctaccagagaagacagttggggtttgaagaagtctcagagctgcagggggaccccggctacccactcgggcggtttggagaagccatcactgctctgacagacatcaacggcgatgggctggtagacgtggctgtgggggcccctctggaggagcagggggctgtgtacatcttcaatgggaggcacggggggcttagtccccagccaagtcagcggatagaagggacccaagtgctctcaggaattcagtggtttggacgctccatccatggggtgaaggaccttgaaggggatggcttggcagatgtggctgtgggggctgagagccagatgatcgtgctgagctcccggcccgtggtggatatggtcaccctgatgtccttctctccagctgagatcccagtgcatgaagtggagtgctcctattcaaccagtaacaagatgaaagaaggagttaatatcacaatctgtttccagatcaagtctctcatcccccagttccaaggccgcctggttgccaatctcacttacactctgcagctggatggccaccggaccagaagacgggggttgttcccaggagggagacatgaactcagaaggaatatagctgtcaccaccagcatgtcatgcactgacttctcatttcatttcccggtatgtgttcaagacctcatctcccccatcaatgtttccctgaatttctctctttgggaggaggaagggacaccgagggaccaaagggcgcagggcaaggacataccgcccatcctgagaccctccctgcactcggaaacctgggagatcccttttgagaagaactgtggggaggacaagaagtgtgaggcaaacttgagagtgtccttctctcctgcaagatccagagccctgcgtctaactgcttttgccagcctctctgtggagctgagcctgagtaacttggaagaagatgcttactgggtccagctggacctgcacttccccccgggactctccttccgcaaggtggagatgctgaagccccatagccagatacctgtgagctgcgaggagcttcctgaagagtccaggcttctgtccagggcattatcttgcaatgtgagctctcccatcttcaaagcaggccactcggttgctctgcagatgatgtttaatacactggtaaacagctcctggggggactcggttgaattgcacgccaatgtgacctgtaacaatgaggactcagacctcctggaggacaactcagccactaccatcatccccatcctgtaccccatcaacatcctcatccaggaccaagaagactccacactctatgtcagtttcacccccaaaggccccaagatccaccaagtcaagcacatgtaccaggtgaggatccagccttccatccacgaccacaacatacccaccctggaggctgtggttggggtgccacagcctcccagcgaggggcccatcacacaccagtggagcgtgcagatggagcctcccgtgccctgccactatgaggatctggagaggctcccggatgcagctgagccttgtctccccggagccctgttccgctgccctgttgtcttcaggcaggagatcctcgtccaagtgatcgggactctggagctggtgggagagatcgaggcctcttccatgttcagcctctgcagctccctctccatctccttcaacagcagcaagcatttccacctctatggcagcaacgcctccctggcccaggttgtcatgaaggttgacgtggtgtatgagaagcagatgctctacctctacgtgctgagcggcatcggggggctgctgctgctgctgctcattttcatagtgctgtacaaggttggtttcttcaaacggaacctgaaggagaagatggaggctggcagaggtgtcccgaatggaatccctgcagaagactctgagcagctggcatctgggcaagaggctggggatcccggctgcctgaagcccctccatgagaaggactctgagagtggtggtggcaaggactgagtccaggcctgtgaggtgcagagtgcccagaactggactcaggatgcccagggccactctgcctctgcctgcattctgccgtgtgccctcgggcgagtcactgcctctccctggccctcagtttccctatctcgaacatggaactcattcctgcctgtctcctttgcaggctcatagggaagacctgctgagggaccagccaagagggctgcaaaagtgagggcttgtcattaccagacggttcaccagcctctcttggtttccttccttggaagagaatgtctgatctaaatgtggagaaactgtagtctcaggacctagggatgttctggccctcacccctgccctgggatgtccacagatgcctccaccccccagaacctgtccttgcacactcccctgcactggagtccagtctcttctgctggcagaaagcaaatgtgacctgtgtcactacgtgactgtggcacacgccttgttcttggccaaagaccaaattccttggcatgccttccagcaccctgcaaaatgagaccctcgtggccttccccagcctcttctagagccgtgatgcctccctgttgaagctctggtgacaccagcctttctcccaggccaggctccttcctgtcttcctgcattcacccagacagctccctctgcctgaaccttccatctcgccacccctccttccttgaccagcagatcccagctcacgtcacacttggttgggtcctcacatctttcacacttccaccagcctgcactactccctcaaagcacacgtcatgtttcttcatccggcagcctggatgttttttccctgtttaatgattgacgtacttagcagctatctctcagtgaactgtgagggtaaaggctatacttgtcttgttcaccttgggatgatgcctcatgatatgtcagggcgtgggacatctagtaggtgcttgacataatttcactgaattaatgacagagccagtgggaagatacagaaaaagaggggctgggctgggcgcggtggttcacgcctgtaatcccagcactttgggaggccaaggagggtggatcacctgaggtcaggagttagaggccagcctggcgaaaccccatctctactaaaaatacaaaatccaggcgtggtggcacacacctgtagtcccagctactcaggaggttgaggtaggagaattgcttgaacctgggaggtggaggttgcagtgagccaagattgcgccattgcactccagcctgggcaacacagcgagactccgtctcaaggaaaaaataaaaataaaaagcgggcacgggcccgtgacatccccacccttggaggctgtcttctcaggctctgccctgccctagctccacaccctctcccaggacccatcacgcctgtgcagtggcccccacagaaagactgagctcaaggtgggaaccacgtctgctaacttggagccccagtgccaagcacagtgcctgcatgtatttatccaataaatgtgaaattctgtcca

SEQ ID NO: 44 - RNA, 913 nt, synthetic construct
  source 1..913: mol_type = other RNA
aaagcgagcgacatgtccctttggggagcagtccctctgcaccccagagtgaggaggacgcaggggtcagaggtggctacagggcaggcagaggaggcacctgtagggggtggtgggctggtggcccaggagaagtcaggaagggagcccagctggtgacaagagagcccagaggtgcctggggctgagtgtgagagcccggaagatttcagccatgcctcacagctccgacagcagtgactccagcttcagccgctctcctccccctggcaaacaggactcatctgatgatgtgagaagagttcagaggagggagaaaaatcgtattgccgcccagaagagccgacagaggcagacacagaaggccgacaccctgcacctggagagcgaagacctggagaaacagaacgcggctctacgcaaggagatcaagcagctcacagaggaactgaagtacttcacgtcggtgctgaacagccacgagcccctgtgctcggtgctggccgccagcacgccctcgccccccgaggtggtgtacagcgcccacgcattccaccaacctcatgtcagctccccgcgcttccagccctgagcttccgatgcggggagagcagagcctcgggaggggcacacagactgtggcagagctgcgcccatcccgcagaggcccctgtccacctggagacccggagacagaggcctggacaaggagtgaacacgggaactgtcacgactggaagggcgtgaggcctcccagcagtgccgcagcgtttcgaggggcgtgtgctggaccccaccactgtgggttgcaggcccaatgcagaagagtattaagaaagatgctcaagtcccatggcacagagcaaggcgggcagggaacggttatttttctaaataaatgctttaaaagaaa

SEQ ID NO: 45 - RNA, 6075 nt, synthetic construct
  source 1..6075: mol_type = other RNA
ggtgtgacttaggacggggcgatggcggctgagaggagctgcgcgtgcgcgaacatgtaactggtgggatctgcggcggctcccagatgatggtcgtcctcctgggcgcgacgaccctagtgctcgtcgccgtggcgccatgggtgttgtccgcagccgcaggtggaaaaaatctaaaatctcctcaaaaagtagaggtcgacatcatagatgacaactttatcctgaggtggaacaggagcgatgagtctgtcgggaatgtgactttttcattcgattatcaaaaaactgggatggataattggataaaattgtctgggtgtcagaatattactagtaccaaatgcaacttttcttcactcaagctgaatgtttatgaagaaattaaattgcgtataagagcagaaaaagaaaacacttcttcatggtatgaggttgactcatttacaccatttcgcaaagctcagattggtcctccagaagtacatttagaagctgaagataaggcaatagtgatacacatctctcctggaacaaaagatagtgttatgtgggctttggatggtttaagctttacatatagcttagttatctggaaaaactcttcaggtgtagaagaaaggattgaaaatatttattccagacataaaatttataaactctcaccagagactacttattgtctaaaagttaaagcagcactacttacgtcatggaaaattggtgtctatagtccagtacattgtataaagaccacagttgaaaatgaactacctccaccagaaaatatagaagtcagtgtccaaaatcagaactatgttcttaaatgggattatacatatgcaaacatgacctttcaagttcagtggctccacgcctttttaaaaaggaatcctggaaaccatttgtataaatggaaacaaatacctgactgtgaaaatgtcaaaactacccagtgtgtctttcctcaaaacgttttccaaaaaggaatttaccttctccgcgtacaagcatctgatggaaataacacatctttttggtctgaagagataaagtttgatactgaaatacaagctttcctacttcctccagtctttaacattagatcccttagtgattcattccatatctatatcggtgctccaaaacagtctggaaacacgcctgtgatccaggattatccactgatttatgaaattattttttgggaaaacacttcaaatgctgagagaaaaattatcgagaaaaaaactgatgttacagttcctaatttgaaaccactgactgtatattgtgtgaaagccagagcacacaccatggatgaaaagctgaataaaagcagtgtttttagtgacgctgtatgtgagaaaacaaaaccaggaaatacctctaaaatttggcttatagttggaatttgtattgcattatttgctctcccgtttgtcatttatgctgcgaaagtcttcttgagatgcatcaattatgtcttctttccatcacttaaaccttcttccagtatagatgagtatttctctgaacagccattgaagaatcttctgctttcaacttctgaggaacaaatcgaaaaatgtttcataattgaaaatataagcacaattgctacagtagaagaaactaatcaaactgatgaagatcataaaaaatacagttcccaaactagccaagattcaggaaattattctaatgaagatgaaagcgaaagtaaaacaagtgaagaactacagcaggactttgtatgaccagaaatgaactgtgtcaagtataaggtttttcagcaggagttacactgggagcctgaggtcctcaccttcctctcagtaactacagagaggacgtttccctgtttagggaaagaaaaaacatcttcagatcataggtcctaaaaatacgggcaagctcttaactatttaaaaatgaaattacaggcccgggcacggtggctcacacctgtaatcccagcactttgggaggctgaggcaggcagatcatgaggtcaagagatcgagaccagcctggccaacgtggtgaaaccccatctctactaaaaatacaaaaattagccgggtgtggtggcgcgcgcctgttgtcttagctactcaggaggctgaggcaggagaatcgcttgaaaacaggaggtggaggttgcagtgagccgagatcacgccactgcactccagcctggtgacagcgtgagactctttaaaaaaagaaattaaaagagttgagacaaacgtttcctacattcttttccatgtgtaaaatcatgaaaaagcctgtcaccggacttgcattggatgagatgagtcagaccaaaacagtggccacccgtcttcctcctgtgagcctaagtgcagccgtgctagctgcgcaccgtggctaaggatgacgtctgtgttcctgtccatcactgatgctgctggctactgcatgtgccacacctgtctgttcgccattcctaacattctgtttcattcttcctcgggagatatttcaaacatttggtcttttcttttaacactgagggtaggcccttaggaaatttatttaggaaagtctgaacacgttatcacttggttttctggaaagtagcttaccctagaaaacagctgcaaatgccagaaagatgatccctaaaaatgttgagggacttctgttcattcatcccgagaacattggcttccacatcacagtatctacccttacatggtttaggattaaagccaggcaatcttttactatgcattaagacctctgattcaaaacttattagaacagtagcttctgctggaatttgcaatcactgaagtcatagaaaataggtaactatctaattagagaaataattgttgtattttaagatctgagagtgtgtacaagttttagtatacatgccatgccagaagatagtgtatgcaagaagtcttgggaccagaaaatggcaatgataggagactgacatagaagaagaatgcttccctaggaaaaaggtcgctggctttggtgcaagaggaagaagaatgttccactggaagcctgagcacctaatcagctctcagtgatcaacccactcttgttatgggtggtctctgtcactttgaatgccaggctggcttctcgtctagcagtattcagataccccttctgctcagcctgcttggcgttaaaatacaaatcattgaactgagggggaaaaatgtaactaggaagaaaaacccaatttaagaaattacataatgctttccaaaggcacctacaacttagttttaaattacttgctactggggattacccatggatatccttaataggcaggaagtctgggaattctggtggcctctagggcagtgttctcacagcaccgttccgacagggaccagtgaaagaaaagagacaaagttagaacgtgctggggagcggccatttctaaggccagtctggtttaagtagtcatttctgctgaaaaaacagatgatcctggtggaagaaaaggttgaaggcagctgccctcgggagggctgtgatgctcggcacatcctgcctggcacatacacgtgtctgcaggccacaccgtgcatgtccccagacctgccgcctggcttctggagtgcttcaagcagagcatggtgggtcattgaggagacccaggaatctcatctgagaacccactctctgccggagaaccccatggtgacacattttcatctttctgaccagaggctgtttttttttttttttgagacagtctcattctgttgcccaggctggagtgcagtggcttgatctcggctcactgcaacctcgcctcccgggttcaagcaattctctgccgcagcctccagagtagctgggataacaggtgcccaccaccacaccccactaatttttgtatttgtatttttagtagagatggggtttcaccatgttggtcaggctggtcttggactcctgacctcatgctccacccgcttcggcctcccaaagttctgggattacaggtgtgagccaccgtgcacggccggcctgacctttggaaaagccttgtcactttggacgtttgcgtctttgaagaggcgatgggagcatatcatgactgcctgccaccattgcttttcagactaccacaactcaatcatgctgtccaggacttctggccctgtgttcaccactgggaaaacgtacttcagactggatagcctaaaaaggagcaatgcccttgtaggatgtggagaagggaaaatacggacattaacattaaaagacaccagtgaaattgttaggtctctaggaagttggagcacaaggcttcacgctttaagaccatctgtggttttcagtgaacaagcgctgagcaccagcagcagaaaacaacaacaaaaaaacacctcgtttttaccttgtcttctagacatgaaaaggcagttgcattccactctgcattatgttctacatgttgctttatcagtatatgcttagctgtaagtgacaagtattttttctgaacagaagtttacttagaaataccatgcacttgggggtaccaattaaccgcctgaaaattagcatattgatagttcttagagagaccagatataatctaagaatttatatgaaagatttgtatcattagagccagaaataattttatattaatatataatacagattaacattatatataatatgtacctgtgtcacttctgacatgagcctgtaaacatatattcatatatgtacctgcacatgtacccacctgatgtaggtcttattcctttagtatggacttaaagtacttattcatataccttgtaactaaaaattagaacagctccctagaattgtgaacttttaagagtctgactagaaatttgcaacttataaaaaagttacttttaaaaatataagttagggctaggcacagtggctcatgcctataatctcagcacttttgggaggccaagacaggaggatcacttcaggccaggagttcaagatcaaccaacctgggtaacatggccagaccccatctctatttatatatatatatataaaacttagagtttttatcttcccctaaaagaggccgtgatatttgcagcagcctcaaattgctcttaaggggtttaggtgtgcagaagctttcctttccctacccagtaaccatgtgactactaacgtggtatattgatttattttgtttgctgtctgtctcccctgccccactgctggaacagaggctccaagaaaacagggaccttattattcattactgcatccccagtaatgaaagtacttagaaaataattattgaatgaatgaaatctaaactgtgaacctgagggtgtttgtggcagtgtttgttttactgaattgtagaaggacataaccgtgttttcagtgtttctatggaacaaacttgtacattttatttcacttgtgttttgtcttaaaccctactgctggaaacaattttatgtaataagcaatgggcccaaaagtctaggagtttttttgtacttagtgaatttgtatgcaacagagatgctgcagctgatgcctttaaaaggtattcatcatggaagagctgaggcctgtgcttggtgttccagagcccagggttgagcatcctgaaggagccactgcagccgtcactgtccccagagcctgtggagatagagcctgtttgctgctttttcttcccgctcttaagacatggctggagctcagtcttcattgaatgaagtttgctgtggtattgcatagccttgctttcttgaactaaactgtttgcccttcacaagtagttcttctttcaggattagttcgttccaaggaggctcttcagtctcacagataagtagatctctcctgctgtctggacacatttcactcggaaattgaatacaatttgtattcaggctgggaacctgaacacacacttgtgtttttaagcttcccttttttacagtggacaaggacacaaataataaataaatcatccctaatgcccaagaaatgccctggtacttagtaataacaaaataccagtaacttcca

SEQ ID NO: 46 - RNA, 1735 nt, synthetic construct
  source 1..1735: mol_type = other RNA
ctctgtcagaatggccaccatggtaccatccgtgttgtggcccagggcctgctggactctgctggtctgctgtctgctgaccccaggtgtccaggggcaggagttccttttgcgggtggagccccagaaccctgtgctctctgctggagggtccctgtttgtgaactgcagtactgattgtcccagctctgagaaaatcgccttggagacgtccctatcaaaggagctggtggccagtggcatgggctgggcagccttcaatctcagcaacgtgactggcaacagtcggatcctctgctcagtgtactgcaatggctctcagataacaggctcctctaacatcaccgtgtacaggctcccggagcgtgtggagctggcacccctgcctccttggcagccggtgggccagaacttcaccctgcgctgccaagtggaggatgggtcgccccggaccagcctcacggtggtgctgcttcgctgggaggaggagctgagccggcagcccgcagtggaggagccagcggaggtcactgccactgtgctggccagcagagacgaccacggagcccctttctcatgccgcacagaactggacatgcagccccaggggctgggactgttcgtgaacacctcagccccccgccagctccgaacctttgtcctgcccgtgacccccccgcgcctcgtggccccccggttcttggaggtggaaacgtcgtggccggtggactgcaccctagacgggctttttccagcctcagaggcccaggtctacctggcgctgggggaccagatgctgaatgcgacagtcatgaaccacggggacacgctaacggccacagccacagccacggcgcgcgcggatcaggagggtgcccgggagatcgtctgcaacgtgaccctagggggcgagagacgggaggcccgggagaacttgacggtctttagcttcctaggacccattgtgaacctcagcgagcccaccgcccatgaggggtccacagtgaccgtgagttgcatggctggggctcgagtccaggtcacgctggacggagttccggccgcggccccggggcagccagctcaacttcagctaaatgctaccgagagtgacgacggacgcagcttcttctgcagtgccactctcgaggtggacggcgagttcttgcacaggaacagtagcgtccagctgcgagtcctgtatggtcccaaaattgaccgagccacatgcccccagcacttgaaatggaaagataaaacgagacacgtcctgcagtgccaagccaggggcaacccgtaccccgagctgcggtgtttgaaggaaggctccagccgggaggtgccggtggggatcccgttcttcgtcaacgtaacacataatggtacttatcagtgccaagcgtccagctcacgaggcaaatacaccctggtcgtggtgatggacattgaggctgggagctcccactttgtccccgtcttcgtggcggtgttactgaccctgggcgtggtgactatcgtactggccttaatgtacgtcttcagggagcaccaacggagcggcagttaccatgttagggaggagagcacctatctgcccctcacgtctatgcagccgacagaagcaatgggggaagaaccgtccagagctgagtgacgctgggatccgggatcaaagttggcgggggcttggctgtgccctcagattccgcaccaataaagccttcaaactccctaa

SEQ ID NO: 47 - RNA, 4405 nt, synthetic construct
  source 1..4405: mol_type = other RNA
aagtcgcgaccagagccattggagggcgcggggactgcaaccctaatcagagcccaaatggcgcagtgggaaatgctgcagaatcttgacagcccctttcaggatcagctgcaccagctttactcgcacagcctcctgcctgtggacattcgacagtacttggctgtctggattgaagaccagaactggcaggaagctgcacttgggagtgatgattccaaggctaccatgctattcttccacttcttggatcagctgaactatgagtgtggccgttgcagccaggacccagagtccttgttgctgcagcacaatttgcggaaattctgccgggacattcagcccttttcccaggatcctacccagttggctgagatgatctttaacctccttctggaagaaaaaagaattttgatccaggctcagagggcccaattggaacaaggagagccagttctcgaaacacctgtggagagccagcaacatgagattgaatcccggatcctggatttaagggctatgatggagaagctggtaaaatccatcagccaactgaaagaccagcaggatgtcttctgcttccgatataagatccaggccaaagggaagacaccctctctggacccccatcagaccaaagagcagaagattctgcaggaaactctcaatgaactggacaaaaggagaaaggaggtgctggatgcctccaaagcactgctaggccgattaactaccctaatcgagctactgctgccaaagttggaggagtggaaggcccagcagcaaaaagcctgcatcagagctcccattgaccacgggttggaacagctggagacatggttcacagctggagcaaagctgttgtttcacctgaggcagctgctgaaggagctgaagggactgagttgcctggttagctatcaggatgaccctctgaccaaaggggtggacctacgcaacgcccaggtcacagagttgctacagcgtctgctccacagagcctttgtggtagaaacccagccctgcatgccccaaactccccatcgacccctcatcctcaagactggcagcaagttcaccgtccgaacaaggctgctggtgagactccaggaaggcaatgagtcactgactgtggaagtctccattgacaggaatcctcctcaattacaaggcttccggaagttcaacattctgacttcaaaccagaaaactttgacccccgagaaggggcagagtcagggtttgatttgggactttggttacctgactctggtggagcaacgttcaggtggttcaggaaagggcagcaataaggggccactaggtgtgacagaggaactgcacatcatcagcttcacggtcaaatatacctaccagggtctgaagcaggagctgaaaacggacaccctccctgtggtgattatttccaacatgaaccagctctcaattgcctgggcttcagttctctggttcaatttgctcagcccaaaccttcagaaccagcagttcttctccaacccccccaaggccccctggagcttgctgggccctgctctcagttggcagttctcctcctatgttggccgaggcctcaactcagaccagctgagcatgctgagaaacaagctgttcgggcagaactgtaggactgaggatccattattgtcctgggctgacttcactaagcgagagagccctcctggcaagttaccattctggacatggctggacaaaattctggagttggtacatgaccacctgaaggatctctggaatgatggacgcatcatgggctttgtgagtcggagccaggagcgccggctgctgaagaagaccatgtctggcacctttctactgcgcttcagtgaatcgtcagaagggggcattacctgctcctgggtggagcaccaggatgatgacaaggtgctcatctactctgtgcaaccgtacacgaaggaggtgctgcagtcactcccgctgactgaaatcatccgccattaccagttgctcactgaggagaatatacctgaaaacccactgcgcttcctctatccccgaatcccccgggatgaagcttttgggtgctactaccaggagaaagttaatctccaggaacggaggaaatacctgaaacacaggctcattgtggtctctaatagacaggtggatgaactgcaacaaccgctggagcttaagccagagccagagctggagtcattagagctggaactagggctggtgccagagccagagctcagcctggacttagagccactgctgaaggcagggctggatctggggccagagctagagtctgtgctggagtccactctggagcctgtgatagagcccacactatgcatggtatcacaaacagtgccagagccagaccaaggacctgtatcacagccagtgccagagccagatttgccctgtgatctgagacatttgaacactgagccaatggaaatcttcagaaactgtgtaaagattgaagaaatcatgccgaatggtgacccactgttggctggccagaacaccgtggatgaggtttacgtctcccgccccagccacttctacactgatggacccttgatgccttctgacttctaggaaccacatttcctctgttcttttcatatctcttgcccttcctactcctcatagcatgatattgttctccaaggatgggaatcaggcatgtgtcccttccaagctgtgttaactgttcaaactcaggcctgtgtgactccattggggtgagaggtgaaagcataacatgggtacagaggggacaacaatgaatcagaacagatgctgagccataggtctaaataggatcctggaggctgcctgctgtgctgggaggtataggggtcctgggggcaggccagggcagttgacaggtacttggagggctcagggcagtggcttctttccagtatggaaggatttcaacattttaatagttggttaggctaaactggtgcatactggcattggcccttggtggggagcacagacacaggataggactccatttctttcttccattccttcatgtctaggataacttgctttcttctttcctttactcctggctcaagccctgaatttcttcttttcctgcaggggttgagagctttctgccttagcctaccatgtgaaactctaccctgaagaaagggatggataggaagtagacctctttttcttaccagtctcctcccctactctgcccctaagctggctgtacctgttcctcccccataaaatgatcctgccaatctaatgtgagtgtgaagctttgcacactagtttatgctacctagtctccactttctcaatgcttaggagacagatcactcctggaggctggggatggtaggattgctggggatttttttttttttaaacagggtctcactctgttgcccaggctagagtgcaatggtgcaatcacagctcactgcagcctcaacctcctgggttcaagcaatcctcctacctcagcctcctgggtagctagcaccatggcatgcgccaccatgccctattttttttttttaaagacagggtcttgctatattgcccaggctggtcttgaactgggctcaagtgatcctcacgccttggcctcccaaagtgctgggattataggcatgagccactgtgcttggccaggatttttttttttttttttttgagatggagtttctctcttgttgtccaggctggagtgcaatggtgtgatctcggctcactgcaacctccgccttccgggttcaagtgactctcctgcctcagcctccccagtagctgggattacagatctgcaccaccatgcccagctaattttgtatttttagtagagacggggtttctccatgttggtcaggctggtctcgaactcctgacctcaagtgatctgtccacctcggcctcccagagtgctgggattacaggcgtgagccactgttcccagcaggaatttcttttttatagtattggataaagtttggtgtttttacagaggagaagcaatgggtcttagctctttctctattatgttatcatcctcccttttttgtacaatatgttgtttacctgaaaggaaggtttctattcgttggttgtggacctggacaaagtccaagtctgtggaacttaaaaccttgaaggtctgtcataggactctggacaatctcacaccttagctattcccagggaaccccagggggcaactgacattgctccaagatgttctcctgatgtagcttgagatataaaggaaaggccctgcacaggtggctgtttcttgtctgttatgtcagaggaacagtcctgttcagaaaggggctcttctgagcagaaatggctaataaactttgtgctgatctggaaa

SEQ ID NO: 48 - RNA, 1369 nt, synthetic construct
  source 1..1369: mol_type = other RNA
ctcttttccgtggcgcctcggaggcgttcagctgcttcaagatgaagctgaacatctccttcccagccactggctgccagaaactcattgaagtggacgatgaacgcaaacttcgtactttctatgagaagcgtatggccacagaagttgctgctgacgctctgggtgaagaatggaagggttatgtggtccgaatcagtggtgggaacgacaaacaaggtttccccatgaagcagggtgtcttgacccatggccgtgtccgcctgctactgagtaaggggcattcctgttacagaccaaggagaactggagaaagaaagagaaaatcagttcgtggttgcattgtggatgcaaatctgagcgttctcaacttggttattgtaaaaaaaggagagaaggatattcctggactgactgatactacagtgcctcgccgcctgggccccaaaagagctagcagaatccgcaaacttttcaatctctctaaagaagatgatgtccgccagtatgttgtaagaaagcccttaaataaagaaggtaagaaacctaggaccaaagcacccaagattcagcgtcttgttactccacgtgtcctgcagcacaaacggcggcgtattgctctgaagaagcagcgtaccaagaaaaataaagaagaggctgcagaatatgctaaacttttggccaagagaatgaaggaggctaaggagaagcgccaggaacaaattgcgaagagacgcagactttcctctctgcgagcttctacttctaagtctgaatccagtcagaaataagattttttgagtaacaaataaataagatcagactctgatctctgttgacttttcattgctgatagaaaactacataaatgaagagagggaaagttaggtcatagaaaatggggatatgtatatatggtattccaatggtggataaagtcagacctattgtgtgtggtagtggaagacaaggtcagtgtacaggggttcctttcaggggatgggtggcacaggaagggattctgagcataagacacctgcctcttcagaatggcatggaacttaggggaaatgatgaggactattaatcttttttatatagtttatttttgaggaatatagctctttaaagcactatacacaatttaatacatgaaaattgaccttgtgaagatgaacatgtcttttttaaaaggtaacttttaaggcatagttttagtggatacctagttttagtggataccatccactaaatggtttttaagccatttcaaatttgttttaacaaagcttttcaactccagtgaattgttaggctgttcacacactgaaaaggaaatgactaaaaacattcttggatcagtgaaaaa

SEQ ID NO: 49 - RNA, 977 nt, synthetic construct
  source 1..977: mol_type = other RNA
gcagacagcggcgggcgcaggacgtgcactatggctcggggctcgctgcgccggttgctgcggctcctcgtgctggggctctggctggcgttgctgcgctccgtggccggggagcaagcgccaggcaccgccccctgctcccgcggcagctcctggagcgcggacctggacaagtgcatggactgcgcgtcttgcagggcgcgaccgcacagcgacttctgcctgggctgcgctgcagcacctcctgcccccttccggctgctttggcccatccttgggggcgctctgagcctgaccttcgtgctggggctgctttctggctttttggtctggagacgatgccgcaggagagagaagttcaccacccccatagaggagaccggcggagagggctgcccagctgtggcgctgatccagtgacaatgtgccccctgccagccggggctcgcccactcatcattcattcatccattctagagccagtctctgcctcccagacgcggcgggagccaagctcctccaaccacaaggggggtggggggcggtgaatcacctctgaggcctgggcccagggttcaggggaaccttccaaggtgtctggttgccctgcctctggctccagaacagaaagggagcctcacgctggctcacacaaaacagctgacactgactaaggaactgcagcatttgcacaggggaggggggtgccctccttcctagaggccctgggggccaggctgacttggggggcagacttgacactaggccccactcactcagatgtcctgaaattccaccacgggggtcaccctggggggttagggacctatttttaacactagggggctggcccactaggagggctggccctaagatacagacccccccaactccccaaagcggggaggagatatttattttggggagagtttggaggggagggagaatttattaataaaagaatctttaactttaaa

SEQ ID NO: 50 - RNA, 2117 nt, synthetic construct
  source 1..2117: mol_type = other RNA
gaggtgtgagcagctgccgaagtcagttccttgtggagccggagctgggcgcggattcgccgaggcaccgaggcactcagaggaggcgccatgtcagaaccggctggggatgtccgtcagaacccatgcggcagcaaggcctgccgccgcctcttcggcccagtggacagcgagcagctgagccgcgactgtgatgcgctaatggcgggctgcatccaggaggcccgtgagcgatggaacttcgactttgtcaccgagacaccactggagggtgacttcgcctgggagcgtgtgcggggccttggcctgcccaagctctaccttcccacggggccccggcgaggccgggatgagttgggaggaggcaggcggcctggcacctcacctgctctgctgcaggggacagcagaggaagaccatgtggacctgtcactgtcttgtacccttgtgcctcgctcaggggagcaggctgaagggtccccaggtggacctggagactctcagggtcgaaaacggcggcagaccagcatgacagatttctaccactccaaacgccggctgatcttctccaagaggaagccctaatccgcccacaggaagcctgcagtcctggaagcgcgagggcctcaaaggcccgctctacatcttctgccttagtctcagtttgtgtgtcttaattattatttgtgttttaatttaaacacctcctcatgtacataccctggccgccccctgccccccagcctctggcattagaattatttaaacaaaaactaggcggttgaatgagaggttcctaagagtgctgggcatttttattttatgaaatactatttaaagcctcctcatcccgtgttctccttttcctctctcccggaggttgggtgggccggcttcatgccagctacttcctcctccccacttgtccgctgggtggtaccctctggaggggtgtggctccttcccatcgctgtcacaggcggttatgaaattcaccccctttcctggacactcagacctgaattctttttcatttgagaagtaaacagatggcactttgaaggggcctcaccgagtgggggcatcatcaaaaactttggagtcccctcacctcctctaaggttgggcagggtgaccctgaagtgagcacagcctagggctgagctggggacctggtaccctcctggctcttgatacccccctctgtcttgtgaaggcagggggaaggtggggtcctggagcagaccaccccgcctgccctcatggcccctctgacctgcactggggagcccgtctcagtgttgagccttttccctctttggctcccctgtaccttttgaggagccccagctaccctttttctccagctgggctctgcaattcccctctgctgctgtccctcccccttgtcctttcccttcagtaccctctcagctccaggtggctctgaggtgcctgtcccacccccacccccagctcaatggactggaaggggaagggacacacaagaagaagggcaccctagttctacctcaggcagctcaagcagcgaccgccccctcctctagctgtgggggtgagggtcccatgtggtggcacaggcccccttgagtggggttatctctgtgttaggggtatatgatgggggagtagatctttctaggagggagacactggcccctcaaatcgtccagcgaccttcctcatccaccccatccctccccagttcattgcactttgattagcagcggaacaaggagtcagacattttaagatggtggcagtagaggctatggacagggcatgccacgtgggctcatatggggctgggagtagttgtctttcctggcactaacgttgagcccctggaggcactgaagtgcttagtgtacttggagtattggggtctgaccccaaacaccttccagctcctgtaacatactggcctggactgttttctctcggctccccatgtgtcctggttcccgtttctccacctagactgtaaacctctcgagggcagggaccacaccctgtactgttctgtgtctttcacagctcctcccacaatgctgaatatacagcaggtgctcaataaatgattcttagtgacttta

SEQ ID NO: 51 - RNA, 2799 nt, synthetic construct
  source 1..2799: mol_type = other RNA
agagggatgcgggcggcagagctcgagaggcggctgccgggctgcggggcgccttgactctccctccaccctgcctcctcgggctccactcgtctgcccctggactcccgtctcctcctgtcctccggcttcccagagctccctccttatggcagcagcttcccgcgtctccggcgcagcttctcagcggacgaccctctcgctccggggctgagcccagtccctggatgttgctgaaactctcgagatcatgcgcgggtttggctgctgcttccccgccgggtgccactgccaccgccgccgcctctgctgccgccgtccgcgggatgctcagtagcccgctgcccggcccccgcgatcctgtgttcctcggaagccgtttgctgctgcagagttgcacgaactagtcatggtgctgtgggagtccccgcggcagtgcagcagctggacactttgcgagggcttttgctggctgctgctgctgcccgtcatgctactcatcgtagcccgcccggtgaagctcgctgctttccctacctccttaagtgactgccaaacgcccaccggctggaattgctctggttatgatgacagagaaaatgatctcttcctctgtgacaccaacacctgtaaatttgatggggaatgtttaagaattggagacactgtgacttgcgtctgtcagttcaagtgcaacaatgactatgtgcctgtgtgtggctccaatggggagagctaccagaatgagtgttacctgcgacaggctgcatgcaaacagcagagtgagatacttgtggtgtcagaaggatcatgtgccacagatgcaggatcaggatctggagatggagtccatgaaggctctggagaaactagtcaaaaggagacatccacctgtgatatttgccagtttggtgcagaatgtgacgaagatgccgaggatgtctggtgtgtgtgtaatattgactgttctcaaaccaacttcaatcccctctgcgcttctgatgggaaatcttatgataatgcatgccaaatcaaagaagcatcgtgtcagaaacaggagaaaattgaagtcatgtctttgggtcgatgtcaagataacacaactacaactactaagtctgaagatgggcattatgcaagaacagattatgcagagaatgctaacaaattagaagaaagtgccagagaacaccacataccttgtccggaacattacaatggcttctgcatgcatgggaagtgtgagcattctatcaatatgcaggagccatcttgcaggtgtgatgctggttatactggacaacactgtgaaaaaaaggactacagtgttctatacgttgttcccggtcctgtacgatttcagtatgtcttaatcgcagctgtgattggaacaattcagattgctgtcatctgtgtggtggtcctctgcatcacaaggaaatgccccagaagcaacagaattcacagacagaagcaaaatacagggcactacagttcagacaatacaacaagagcgtccacgaggttaatctaaagggagcatgtttcacagtggctggactaccgagagcttggactacacaatacagtattatagacaaaagaataagacaagagatctacacatgttgccttgcatttgtggtaatctacaccaatgaaaacatgtactacagctatatttgattatgtatggatatatttgaaatagtatacattgtcttgatgttttttctgtaatgtaaataaactatttatatcacacaatatagttttttctttcccatgtatttgttatatataataaatactcagtgatgagaaaaaattggcattcttaaatttgcggtatctcataactgtaaatataatcagactagtacaatctgtacagctaccaatatttcatgtttcttctcatcttgagacagcacattagttcgtacaggactcagtggctaggttttgaatgattccaagatcaagggaaatgatggttattggaaaagagaaaaaataatttactttatatcgagtgaggataaaatatttccgatctttgaatcatctctatttcatcaactttcttccctggtcttccattttcatccctagagcagaaaaatctctggcatataaactaaataaaagaagaaggggagggaaagtgttttataactcataaaggagagggaaagaaaatattggtttttattggggaagtagcttagaatcccccagttaagtgcatatatctgaacttactgaacaagttacatactaggtatacacagagtggcaaaatatattccatttaggtgggtggaattaccaggggaaaaatgtaataacaccactagatgtgaaacaccaaaatcgtgaattctcaaaagcaccatacaatatgtatagtatatagttctttgaaaagaagttagaatcacaaccaataccccatgaatagctttgtggctaatgcagcaccataatttgtaatggaactaagatgatgatgacgatatttcatgaaaacagagagatgttttgagcatatttatgtggtgaggtaagaaagaaaattaatcctatagcatctgaaagacctcactgggaagttggtatggatttttgtttgatttgtgcatacaaataggtatcacaacttgatctggaaaaaataagctgtgaaaattctcaaggaataagatgaaaataaatcaattattatcatttagctctgcaaagctttccatggctaacacagtaaatttaaataaagctctctttgtctccttcaaa

SEQ ID NO: 52 - RNA, 1017 nt, synthetic construct
  source 1..1017: mol_type = other RNA
agtgccccaggcggcgaggagagcggtgccttgcagggatgctgcgggcgggagcaccaaccggggacttaccccgggcgggagaagtccacaccgggaccaccatcatggcagtggagtttgacgggggcgttgtgatgggttctgattcccgagtgtctgcaggcgaggcggtggtgaaccgagtgtttgacaagctgtccccgctgcacgagcgcatctactgtgcactctctggttcagctgctgatgcccaagccgtggccgacatggccgcctaccagctggagctccatgggatagaactggaggaacctccacttgttttggctgctgcaaatgtggtgagaaatatcagctataaatatcgagaggacttgtctgcacatctcatggtagctggctgggaccaacgtgaaggaggtcaggtatatggaaccctgggaggaatgctgactcgacagccttttgccattggtggctccggcagcacctttatctatggttatgtggatgcagcatataagccaggcatgtctcccgaggagtgcaggcgcttcaccacagacgctattgctctggccatgagccgggatggctcaagcgggggtgtcatctacctggtcactattacagctgccggtgtggaccatcgagtcatcttgggcaatgaactgccaaaattctatgatgagtgaaccttccccagacttctctttcttattttgtaataaactctctagggccaaaacctggtatggtcattgggaaatgagtgctcagggagatggagcttaggggaggtgggtgcttccctcctagatgtcagcatacactctttcttcttttgtcccaggtctaaaacatctttcctagagaaaacaaaagggactaaactagaaatataaagagccctatacatgacaggtgatcacgtactgaatgattttgaagtagtacaaacaataaaaattctcattccgcatcatcatgcggtccatgatgatgaggccgcaa

SEQ ID NO: 53 - RNA, 1542 nt, synthetic construct
  source 1..1542: mol_type = other RNA
acattctccccagaggccgagatgcgggtcatggcgccccgagccctcctcctgctgctctcgggaggcctggccctgaccgagacctgggcctgctcccactccatgaggtatttcgacaccgccgtgtcccggcccggccgcggagagccccgcttcatctcagtgggctacgtggacgacacgcagttcgtgcggttcgacagcgacgccgcgagtccgagaggggagccgcgggcgccgtgggtggagcaggaggggccggagtattgggaccgggagacacagaagtacaagcgccaggcacaggctgaccgagtgagcctgcggaacctgcgcggctactacaaccagagcgaggacgggtctcacaccctccagaggatgtctggctgcgacctggggcccgacgggcgcctcctccgcgggtatgaccagtccgcctacgacggcaaggattacatcgccctgaacgaggacctgcgctcctggaccgccgcggacaccgcggctcagatcacccagcgcaagttggaggcggcccgtgcggcggagcagctgagagcctacctggagggcacgtgcgtggagtggctccgcagatacctggagaacgggaaggagacgctgcagcgcgcagaacccccaaagacacacgtgacccaccaccccctctctgaccatgaggccaccctgaggtgctgggccctgggcttctaccctgcggagatcacactgacctggcagcgggatggggaggaccagacccaggacaccgagcttgtggagaccaggccagcaggagatggaaccttccagaagtgggcagctgtggtggtgccttctggacaagagcagagatacacgtgccatatgcagcacgaggggctgcaagagcccctcaccctgagctgggagccatcttcccagcccaccatccccatcatgggcatcgttgctggcctggctgtcctggttgtcctagctgtccttggagctgtggtcaccgctatgatgtgtaggaggaagagctcaggtggaaaaggagggagctgctctcaggctgcgtgcagcaacagtgcccagggctctgatgagtctctcatcacttgtaaagcctgagacagctgcctgtgtgggactgagatgcaggatttcttcacacctctcctttgtgacttcaagagcctctggcatctctttctgcaaaggcacctgaatgtgtctgcgttcctgttagcataatgtgaggaggtggagagacagcccacccccgtgtccaccgtgacccctgtccccacactgacctgtgttccctccccgatcatctttcctgttccagagaggtggggctggatgtctccatctctgtctcaaattcatggtgcactgagctgcaacttcttacttccctaatgaagttaagaacctgaatataaatttgtgttctcaaatatttgctatgaagcgttgatggattaattaaataagtcaattcctagaagttgagagagcaaataaagacctgagaaccttccagaa

SEQ ID NO: 54 - RNA, 2091 nt, synthetic construct
  source 1..2091: mol_type = other RNA
gagacaggtggtggctacgacggcgaagggagctgagactgtccaggcagccaggttaggccaggaggaccatgtgaatggggccagagggctcccgggctgggcagggaccatgggctgtggctgcagctcacacccggaagatgactggatggaaaacatcgatgtgtgtgagaactgccattatcccatagtcccactggatggcaagggcacgctgctcatccgaaatggctctgaggtgcgggacccactggttacctacgaaggctccaatccgccggcttccccactgcaagacaacctggttatcgctctgcacagctatgagccctctcacgacggagatctgggctttgagaagggggaacagctccgcatcctggagcagagcggcgagtggtggaaggcgcagtccctgaccacgggccaggaaggcttcatccccttcaattttgtggccaaagcgaacagcctggagcccgaaccctggttcttcaagaacctgagccgcaaggacgcggagcggcagctcctggcgcccgggaacactcacggctccttcctcatccgggagagcgagagcaccgcgggatcgttttcactgtcggtccgggacttcgaccagaaccagggagaggtggtgaaacattacaagatccgtaatctggacaacggtggcttctacatctcccctcgaatcacttttcccggcctgcatgaactggtccgccattacaccaatgcttcagatgggctgtgcacacggttgagccgcccctgccagacccagaagccccagaagccgtggtgggaggacgagtgggaggttcccagggagacgctgaagctggtggagcggctgggggctggacagttcggggaggtgtggatggggtactacaacgggcacacgaaggtggcggtgaagagcctgaagcagggcagcatgtccccggacgccttcctggccgaggccaacctcatgaagcagctgcaacaccagcggctggttcggctctacgctgtggtcacccaggagcccatctacatcatcactgaatacatggagaatgggagtctagtggattttctcaagaccccttcaggcatcaagttgaccatcaacaaactcctggacatggcagcccaaattgcagaaggcatggcattcattgaagagcggaattatattcatcgtgaccttcgggctgccaacattctggtgtctgacaccctgagctgcaagattgcagactttggcctagcacgcctcattgaggacaacgagtacacagccagggagggggccaagtttcccattaagtggacagcgccagaagccattaactacgggacattcaccatcaagtcagatgtgtggtcttttgggatcctgctgacggaaattgtcacccacggccgcatcccttacccagggatgaccaacccggaggtgattcagaacctggagcgaggctaccgcatggtgcgccctgacaactgtccagaggagctgtaccaactcatgaggctgtgctggaaggagcgcccagaggaccggcccacctttgactacctgcgcagtgtgctggaggacttcttcacggccacagagggccagtaccagcctcagccttgagaggccttgagaggccctggggttctccccctttctctccagcctgacttggggagatggagttcttgtgccatagtcacatggcctatgcacatatggactctgcacatgaatcccacccacatgtgacacatatgcaccttgtgtctgtacacgtgtcctgtagttgcgtggactctgcacatgtcttgtacatgtgtagcctgtgcatgtatgtcttggacactgtacaaggtacccctttctggctctcccatttcctgagaccacagagagaggggagaagcctgggattgacagaagcttctgcccacctacttttctttcctcagatcatccagaagttcctcaagggccaggactttatctaatacctctgtgtgctcctccttggtgcctggcctggcacacatcaggagttcaataaatgtctgttgatgactgttgta

SEQ ID NO: 55 - RNA, 3691 nt, synthetic construct
  source 1..3691: mol_type = other RNA
aggcttctgggatatgacagcattgccttgtgttagctagcaataagaaaagaagctttgtttggattaacatatataccctcttcattctgcatacctattttttccccaataatttgcagcttaggtccgaggacaccacaaactctgcttaaagggcctggaggctctcaaggcatggccagacgctctgtcttgtacttcatcctgctgaatgctctgatcaacaagggccaagcctgcttctgtgatcactatgcatggactcagtggaccagctgctcaaaaacttgcaattctggaacccagagcagacacagacaaatagtagtagataagtactaccaggaaaacttttgtgaacagatttgcagcaagcaggagactagagaatgtaactggcaaagatgccccatcaactgcctcctgggagattttggaccatggtcagactgtgacccttgtattgaaaaacagtctaaagttagatctgtcttgcgtcccagtcagtttgggggacagccatgcactgcgcctctggtagcctttcaaccatgcattccatctaagctctgcaaaattgaagaggctgactgcaagaataaatttcgctgtgacagtggccgctgcattgccagaaagttagaatgcaatggagaaaatgactgtggagacaattcagatgaaagggactgtgggaggacaaaggcagtatgcacacggaagtataatcccatccctagtgtacagttgatgggcaatgggtttcattttctggcaggagagcccagaggagaagtccttgataactctttcactggaggaatatgtaaaactgtcaaaagcagtaggacaagtaatccataccgtgttccggccaatctggaaaatgtcggctttgaggtacaaactgcagaagatgacttgaaaacagatttctacaaggatttaacttctcttggacacaatgaaaatcaacaaggctcattctcaagtcagggggggagctctttcagtgtaccaattttttattcctcaaagagaagtgaaaatatcaaccataattctgccttcaaacaagccattcaagcctctcacaaaaaggattctagttttattaggatccataaagtgatgaaagtcttaaacttcacaacgaaagctaaagatctgcacctttctgatgtctttttgaaagcacttaaccatctgcctctagaatacaactctgctttgtacagccgaatattcgatgactttgggactcattacttcacctctggctccctgggaggcgtgtatgaccttctctatcagtttagcagtgaggaactaaagaactcaggtttaaccgaggaagaagccaaacactgtgtcaggattgaaacaaagaaacgcgttttatttgctaagaaaacaaaagtggaacataggtgcaccaccaacaagctgtcagagaaacatgaaggttcatttatacagggagcagagaaatccatatccctgattcgaggtggaaggagtgaatatggagcagctttggcatgggagaaagggagctctggtctggaggagaagacattttctgagtggttagaatcagtgaaggaaaatcctgctgtgattgactttgagcttgcccccatcgtggacttggtaagaaacatcccctgtgcagtgacaaaacggaacaacctcaggaaagctttgcaagagtatgcagccaagttcgatccttgccagtgtgctccatgccctaataatggccgacccaccctctcagggactgaatgtctgtgtgtgtgtcagagtggcacctatggtgagaactgtgagaaacagtctccagattataaatccaatgcagtagacggacagtggggttgttggtcttcctggagtacctgtgatgctacttataagagatcgagaacccgagaatgcaataatcctgccccccaacgaggagggaaacgctgtgagggggagaagcgacaagaggaagactgcacattttcaatcatggaaaacaatggacaaccatgtatcaatgatgacgaagaaatgaaagaggtcgatcttcctgagatagaagcagattccgggtgtcctcagccagttcctccagaaaatggatttatccggaatgaaaagcaactatacttggttggagaagatgttgaaatttcatgccttactggctttgaaactgttggataccagtacttcagatgcttaccagacgggacctggagacaaggggatgtggaatgccaacggacggagtgcatcaagccagttgtgcaggaagtcctgacaattacaccatttcagagattgtatagaattggtgaatccattgagctaacttgccccaaaggctttgttgttgctgggccatcaaggtacacatgccaggggaattcctggacaccacccatttcaaactctctcacctgtgaaaaagatactctaacaaaattaaaaggccattgtcagctgggacagaaacaatcaggatctgaatgcatttgtatgtctccagaagaagactgtagccatcattcagaagatctctgtgtgtttgacacagactccaacgattactttacttcacccgcttgtaagtttttggctgagaaatgtttaaataatcagcaactccattttctacatattggttcctgccaagacggccgccagttagaatggggtcttgaaaggacaagactttcatccaacagcacaaagaaagaatcctgtggctatgacacctgctatgactgggaaaaatgttcagcctccacttccaaatgtgtctgcctattgcccccacagtgcttcaagggtggaaaccaactctactgtgtcaaaatgggatcatcaacaagtgagaaaacattgaacatctgtgaagtgggaactataagatgtgcaaacaggaagatggaaatactgcatcctggaaagtgtttggcctagcacaattactgctaggcccagcacaatgaacagatttaccatcccgaagaaccaactcctacaaatgagaattcttgcacaaacagcagactggcatgctcaaagttactgacaaaaattattttctgttagtttgagatcattattctcccctgactctcctgtttgggcatgtcttattcagttccagctcatgacgccctgtagcatacccctaggtaccaacttccacagcagtctcgtaaattctcctgttcacattgtacaaaaataatgtgacttctgaggcccttatgtagcctgtgacattaagcattctcgcaattagaaataagaataaaacccataattttcttcaatgagttaataaacagaaatctccagaacctctgaaacacattcttgaagcccagctttcatatcttcattcaacaaataatttctgagtgtgtatacaggatgtcaagtactgaccaaagtcctgagaactcggcagataataaaacagacaaaagcctttgccttcatgaagcatacattcattcaggggtagacacacaaaaaatgaaataaacaggtaaaatatgtagcatgtttgatggtgataattgttttggagaaaatacaacacggaagggtgagtcccatccttaattatcatcttatgcaaggaaatattccataacaataaacatcgctgtaaggatga

SEQ ID NO: 56 - RNA, 1080 nt, synthetic construct
  source 1..1080: mol_type = other RNA
gcatttgtttcaaggctgtgattctcactatactggtcctgaggaaagggcttctgtgaactgcggtttttagtttttattgtggttcttagttctcatgagacccctcttgaggatatgtgcctatctggtgcctctgctctccactagttgagtgaaaggaaggaggtaatttaccaccatgtttggttcctgtttataagatgttttaagaaagatctgaaacagattttctgaagaaagcagaagctctcttcccattatgacttcggaaatcacttatgctgaagtgaggttcaaaaatgaattcaagtcctcaggcatcaacacagcctcttctgcagagacagcctggagctgttgcccaaagaattggaagtcatttagttccaactgctactttatttctactgaatcagcatcttggcaagacagtgagaaggactgtgctagaatggaggctcacctgctggtgataaacactcaagaagagcaggatttcatcttccagaatctgcaagaagaatctgcttattttgtggggctctcagatccagaaggtcagcgacattggcaatgggttgatcagacaccatacaatgaaagttccacattctggcatccacgtgagcccagtgatcccaatgagcgctgcgttgtgctaaattttcgtaaatcacccaaaagatggggctggaatgatgttaattgtcttggtcctcaaaggtcagtttgtgagatgatgaagatccacttatgaactgaacattctccatgaacaggtggttggattggtatctgtcattgtagggatagataataagctcttcttattcatgtgtaagggaggtccatagaatttaggtggtctgtcaactattctacttatgagagaattggtctgtacattgactgattcactttttcataaagtgagcatttattgagcattttttcatgtgccagagcctgtactggaggcccccattgtgcacacatggagagaacatgagtctctcttaatttttatctggttgctaaagaattatttaccaataaaattatatgatgtggtgtctc

SEQ ID NO: 57 - RNA, 3996 nt, synthetic construct
  source 1..3996: mol_type = other RNA
ccagcccggccgggctccgaggcgagaggctgcatggagtggccggcgcggctctgcgggctgtgggcgctgctgctctgcgccggcggcgggggcgggggcgggggcgccgcgcctacggaaactcagccacctgtgacaaatttgagtgtctctgttgaaaacctctgcacagtaatatggacatggaatccacccgagggagccagctcaaattgtagtctatggtattttagtcattttggcgacaaacaagataagaaaatagctccggaaactcgtcgttcaatagaagtacccctgaatgagaggatttgtctgcaagtggggtcccagtgtagcaccaatgagagtgagaagcctagcattttggttgaaaaatgcatctcacccccagaaggtgatcctgagtctgctgtgactgagcttcaatgcatttggcacaacctgagctacatgaagtgttcttggctccctggaaggaataccagtcccgacactaactatactctctactattggcacagaagcctggaaaaaattcatcaatgtgaaaacatctttagagaaggccaatactttggttgttcctttgatctgaccaaagtgaaggattccagttttgaacaacacagtgtccaaataatggtcaaggataatgcaggaaaaattaaaccatccttcaatatagtgcctttaacttcccgtgtgaaacctgatcctccacatattaaaaacctctccttccacaatgatgacctatatgtgcaatgggagaatccacagaattttattagcagatgcctattttatgaagtagaagtcaataacagccaaactgagacacataatgttttctacgtccaagaggctaaatgtgagaatccagaatttgagagaaatgtggagaatacatcttgtttcatggtccctggtgttcttcctgatactttgaacacagtcagaataagagtcaaaacaaataagttatgctatgaggatgacaaactctggagtaattggagccaagaaatgagtataggtaagaagcgcaattccacactctacataaccatgttactcattgttccagtcatcgtcgcaggtgcaatcatagtactcctgctttacctaaaaaggctcaagattattatattccctccaattcctgatcctggcaagatttttaaagaaatgtttggagaccagaatgatgatactctgcactggaagaagtacgacatctatgagaagcaaaccaaggaggaaaccgactctgtagtgctgatagaaaacctgaagaaagcctctcagtgatggagataatttatttttaccttcactgtgaccttgagaagattcttcccattctccatttgttatctgggaacttattaaatggaaactgaaactactgcaccatttaaaaacaggcagctcataagagccacaggtctttatgttgagtcgcgcaccgaaaaactaaaaataatgggcgctttggagaagagtgtggagtcattctcattgaattataaaagccagcaggcttcaaactaggggacaaagcaaaaagtgatgatagtggtggagttaatcttatcaagagttgtgacaacttcctgagggatctatacttgctttgtgttctttgtgtcaacatgaacaaattttatttgtaggggaactcatttggggtgcaaatgctaatgtcaaacttgagtcacaaagaacatgtagaaaacaaaatggataaaatctgatatgtattgtttgggatcctattgaaccatgtttgtggctattaaaactcttttaacagtctgggctgggtccggtggctcacgcctgtaatcccagcaatttgggagtccgaggcgggcggatcactcgaggtcaggagttccagaccagcctgaccaaaatggtgaaacctcctctctactaaaactacaaaaattaactgggtgtggtggcgcgtgcctgtaatcccagctactcgggaagctgaggcaggtgaattgtttgaacctgggaggtggaggttgcagtgagcagagatcacaccactgcactctagcctgggtgacagagcaagactctgtctaaaaaacaaaacaaaacaaaacaaaacaaaaaaacctcttaatattctggagtcatcattcccttcgacagcattttcctctgctttgaaagccccagaaatcagtgttggccatgatgacaactacagaaaaaccagaggcagcttctttgccaagacctttcaaagccattttaggctgttaggggcagtggaggtagaatgactccttgggtattagagtttcaaccatgaagtctctaacaatgtattttcttcacctctgctactcaagtagcatttactgtgtctttggtttgtgctaggcccccgggtgtgaagcacagaccccttccaggggtttacagtctatttgagactcctcagttcttgccacttttttttttaatctccaccagtcatttttcagaccttttaactcctcaattccaacactgatttccccttttgcattctccctccttcccttccttgtagccttttgactttcattggaaattaggatgtaaatctgctcaggagacctggaggagcagaggataattagcatctcaggttaagtgtgagtaatctgagaaacaatgactaattcttgcatattttgtaacttccatgtgagggttttcagcattgatatttgtgcattttctaaacagagatgaggtggtatcttcacgtagaacattggtattcgcttgagaaaaaaagaatagttgaacctatttctctttctttacaagatgggtccaggattcctcttttctctgccataaatgattaattaaatagcttttgtgtcttacattggtagccagccagccaaggctctgtttatgcttttggggggcatatattgggttccattctcacctatccacacaacatatccgtatatatcccctctactcttacttcccccaaatttaaagaagtatgggaaatgagaggcatttcccccaccccatttctctcctcacacacagactcatattactggtaggaacttgagaactttatttccaagttgttcaaacatttaccaatcatattaatacaatgatgctatttgcaattcctgctcctaggggaggggagataagaaaccctcactctctacaggtttgggtacaagtggcaacctgcttccatggccgtgtagaagcatggtgccctggcttctctgaggaagctggggttcatgacaatggcagatgtaaagttattcttgaagtcagattgaggctgggagacagccgtagtagatgttctactttgttctgctgttctctagaaagaatatttggttttcctgtataggaatgagattaattcctttccaggtattttataattctgggaagcaaaacccatgcctccccctagccatttttactgttatcctatttagatggccatgaagaggatgctgtgaaattcccaacaaacattgatgctgacagtcatgcagtctgggagtggggaagtgatcttttgttcccatcctcttcttttagcagtaaaatagctgagggaaaagggagggaaaaggaagttatgggaatacctgtggtggttgtgatccctaggtcttgggagctcttggaggtgtctgtatcagtggatttcccatcccctgtgggaaattagtaggctcatttactgttttaggtctagcctatgtggattttttcctaacatacctaagcaaacccagtgtcaggatggtaattcttattctttcgttcagttaagtttttcccttcatctgggcactgaagggatatgtgaaacaatgttaacatttttggtagtcttcaaccagggattgtttctgtttaacttcttataggaaagcttgagtaaaataaatattgtctttttgtatgtca

SEQ ID NO: 58 - RNA, 8566 nt, synthetic construct
  source 1..8566: mol_type = other RNA
gactcgaactccaccgcggaaaagaaagcctcagaacgttcgttcgctgcgtccccagccggggccgagccctccgcgacgccagccgggccatgggggccgcacgcagcccgccgtccgctgtcccggggcccctgctggggctgctcctgctgctcctgggcgtgctggccccgggtggcgcctccctgcgactcctggaccaccgggcgctggtctgctcccagccggggctaaactgcacggtcaagaatagtacctgcctggatgacagctggattcaccctcgaaacctgaccccctcctccccaaaggacctgcagatccagctgcactttgcccacacccaacaaggagacctgttccccgtggctcacatcgaatggacactgcagacagacgccagcatcctgtacctcgagggtgcagagttatctgtcctgcagctgaacaccaatgaacgtttgtgcgtcaggtttgagtttctgtccaaactgaggcatcaccacaggcggtggcgttttaccttcagccactttgtggttgaccctgaccaggaatatgaggtgaccgttcaccacctgcccaagcccatccctgatggggacccaaaccaccagtccaagaatttccttgtgcctgactgtgagcacgccaggatgaaggtaaccacgccatgcatgagctcaggcagcctgtgggaccccaacatcaccgtggagaccctggaggcccaccagctgcgtgtgagcttcaccctgtggaacgaatctacccattaccagatcctgctgaccagttttccgcacatggagaaccacagttgctttgagcacatgcaccacatacctgcgcccagaccagaagagttccaccagcgatccaacgtcacactcactctacgcaaccttaaagggtgctgtcgccaccaagtgcagatccagcccttcttcagcagctgcctcaatgactgcctcagacactccgcgactgtttcctgcccagaaatgccagacactccagaaccaattccggactacatgcccctgtgggtgtactggttcatcacgggcatctccatcctgctggtgggctccgtcatcctgctcatcgtctgcatgacctggaggctagctgggcctggaagtgaaaaatacagtgatgacaccaaatacaccgatggcctgcctgcggctgacctgatccccccaccgctgaagcccaggaaggtctggatcatctactcagccgaccaccccctctacgtggacgtggtcctgaaattcgcccagttcctgctcaccgcctgcggcacggaagtggccctggacctgctggaagagcaggccatctcggaggcaggagtcatgacctgggtgggccgtcagaagcaggagatggtggagagcaactctaagatcatcgtcctgtgctcccgcggcacgcgcgccaagtggcaggcgctcctgggccggggggcgcctgtgcggctgcgctgcgaccacggaaagcccgtgggggacctgttcactgcagccatgaacatgatcctcccggacttcaagaggccagcctgcttcggcacctacgtagtctgctacttcagcgaggtcagctgtgacggcgacgtccccgacctgttcggcgcggcgccgcggtacccgctcatggacaggttcgaggaggtgtacttccgcatccaggacctggagatgttccagccgggccgcatgcaccgcgtaggggagctgtcgggggacaactacctgcggagcccgggcggcaggcagctccgcgccgccctggacaggttccgggactggcaggtccgctgtcccgactggttcgaatgtgagaacctctactcagcagatgaccaggatgccccgtccctggacgaagaggtgtttgaggagccactgctgcctccgggaaccggcatcgtgaagcgggcgcccctggtgcgcgagcctggctcccaggcctgcctggccatagacccgctggtcggggaggaaggaggagcagcagtggcaaagctggaacctcacctgcagccccggggtcagccagcgccgcagcccctccacaccctggtgctcgccgcagaggagggggccctggtggccgcggtggagcctgggcccctggctgacggtgccgcagtccggctggcactggcgggggagggcgaggcctgcccgctgctgggcagcccgggcgctgggcgaaatagcgtcctcttcctccccgtggaccccgaggactcgccccttggcagcagcacccccatggcgtctcctgacctccttccagaggacgtgagggagcacctcgaaggcttgatgctctcgctcttcgagcagagtctgagctgccaggcccaggggggctgcagtagacccgccatggtcctcacagacccacacacgccctacgaggaggagcagcggcagtcagtgcagtctgaccagggctacatctccaggagctccccgcagccccccgagggactcacggaaatggaggaagaggaggaagaggagcaggacccagggaagccggccctgccactctctcccgaggacctggagagcctgaggagcctccagcggcagctgcttttccgccagctgcagaagaactcgggctgggacacgatggggtcagagtcagaggggcccagtgcatgagggcggctccccagggaccgcccagatcccagctttgagagaggagtgtgtgtgcacgtattcatctgtgtgtacatgtctgcatgtgtatatgttcgtgtgtgaaatgtaggctttaaaatgtaaatgtctggattttaatcccaggcatccctcctaacttttctttgtgcagcggtctggttatcgtctatccccaggggaatccacacagcccgctcccaggagctaatggtagagcgtccttgaggctccattattcgttcattcagcatttattgtgcacctactatgtggcgggcatttgggataccaagataaattgcatgcggcatggccccagccatgaaggaacttaaccgctagtgccgaggacacgttaaacgaacaggatgggccgggcacggtggctcacgcctgtaatcccagcacactgggaggccgaggcaggtggatcactctgaggtcaggagtttgagccagcctggccaacatggtgaaaccccatctccactaaaaatagaaaaattagccgggcatggtgacacatgcctgtagtcctagctacttgggaggctgaggcaggagaattgcttgaatctgggaggcagaggttgcagtgagccgagattgtgccattgcactgcagcctggatgacagagcgagactctatctcaaaaaaaaaaaaaaaaaaagatggtcacgcgggatgtaaacgctgaatgggccaggtgcagtggctcatgcttgtaatcccagcactttgggaaggcgaggcaggtggattgcttgagctcaggagttcaagaccagcctgggcgacatagtgagacctcatctctacctaaatttttttttagtcagtcatggtggcacatgcctgtagtcccagctactcgggaggctgatgccagatgatcacttgagcccaggaggtagaggctgcagtgagctataatggtaccattgcaatccagcctgggcagcagagtgagaccctgtctcaaaaaaaataaaaaagtagaaagatggagtggaagcctgcccagggttgtgagcatgcacgggaaaggcacccaggtcaggggggatccccgaggagatgcctgagctgaaggattgtggttggggaaagcgtagtcccagcaaggaagcagtttgtgggtaagtgctgggaggtgagtggagtgagcttgtcagggagctgctggtggagcctggaggggaaggagggaggcagtgagagagatcggggtggggggtggggggatgtcgccagagctcaggggtggggacagccttgtgcgcatcagtcctgaggcctggggcacctttcgtctgatgagcctctgcatggagagaggctgagggctaaacacagctggatgtcacctgagttcatttataggaagagagaaatgtcgaggtgaaacgtaaaagcatctggcaggaaggtgagtctgaagccctgcacccgcgttccgactatcagtggggagctgttagcacgtaggattcttcagagcagctgggctggagctcccctgagctcaggaagccccagggtgcaagggcaaggaaatgaggggtggtgggtcagtgaagatctgggcagaccttgtgtggggaaggggtgctgctgtgacttcagggtctgaggtccaaagacagcatttgaaaagaggctctgaagccagtgtttgaagaatttgttcctgaagtacctcctgggggtaggctagaggcttctggcttcagggtcctgaagaacacattgaggtgccgtctgacactggaatagggtgcccttcattcctatgcctgagtccttaactatatttccaacctccagtgaggaggagaagattcggaaatgtgacaggagagcaaacaggacagtttgcatgtgtgtgtgcgcacacatacatgtgcgtgaaagattatcaataaaagtgcataaatttgttgatctggtaagagtttctagcaggaaggtcgagccacttactgtaggtcaagaagttgctagttgcggagttttttcttgcagttagactttacctagtggtagcagggccaccaaagctctgtgtcccagatggtgtatggcccataatccacccaacagcagcaaaggaccaggcaaaggagaacaggagcagaagcctcccagccactagccttttgggctcagtctctccaataatcctggagaggggcttcgttgggtctggacacctaccatgcattctgtgacctttccctagcttccaataaataactgtttgacgcccagagtacaggataccacaatgcactcttcctgcgtagagcacatgttcccatctgctcccattcctcaggaaccttgaattctagctctgctggcctttgagcccatgccagtaaatgtcctgatgggcattgcctactatctccagggcagctgcctttgtcctcctaacagctttattggagtacagttcacttaccatacaatccacaattgaccctgcacaatttgatgccggtttagtatagtcacagttcagcagccatcagcacagtcagtcttagagtttactacccccaaaagaaatccagccccccttagtcaccaccccaacctccccatccctaggcacccctaggctactttgatctctgtagacttgcctcttctggacatgacatagagaaaggagtcataaattctccaaggtgtctgtttcttctttaatgtcattccctgtttctcctcacattccctccccatttcctgggcccagtctcacactggtccttgcttaccctaaatgctattaattccatcactctgagtatggtgtttgctgtccgctgaatgccaagagcttcaagagtgtgtgtaaataaagccacacctttatttttgtattattctgaaccatggctaataaattgtttcaccaagaaatgtctctctaagaacaggtgccctccacgctgtgcccctcccacctcttcagctcgtctcctgagtgtgcagaggtggttccggttgggaaagaagcagcggagcatctaaccatgcctgtgtccaggccgattatgcacgcagccaccaacaagctcccaactcccgcgtagagtttcatgactttttcctgcctactatcttgatcctagttttttttttgttttttttttttttaaggaataattactttgattcaaaaccagtttctcttttctgcataggaaggtccttgaaggtgtttagggtctaaaaagggtggtgttcggtctctgaaacatccattcagcagtttgagctgggatctctgaatgcaagggtatgatggatatacttctttcttgcttttgttgtgttttggttttttgtttgtttttaagtcagggtctctctgtcaccaggctgtattacagtggtgcaatcatggctcactgcagcctcgacctcccaggctcaagccatctttccacctcagcctgccagtggctagaactacaggcgtgcaccactgtgcccggctaatttgtgtgtatatattttgtagaaatggggtttcaccatgttgtccaggctggtcacgaactcctgggctcaagccatctgcccgcctcatcctcccaaagtgctgggattataggcctgagcccaccgtgcctggcctttcctgtttatctttgaaaattaaatagggcataagagagaagaagatgtacttacaatgcagtgggtggttttaactctatagcctttgggctctgtggttggtgctccccttcctaaataaatgaggtgtatgcagggccctcttctgccttagcgccctgccagctgggactccagcaaggcccggggcacctgaggacagagtgagatggagggccgctgctccagcagccgggcctgcatcccacaagtcaactgtgtcggacagaggatccttacaaagaagaggcagcagggttgggggctggccagctgctcgtccgccctaggtagcttgctcatctgtaaagtgggtggggcaggagttcccacctcatggggtcctggcaagcctgcagtatccccgagtggcaccagcctgcttctggggcagagcagtttgtgccccctgaggtaccactgatcctctttccctgctattaggtattgctctcttcctccggtgtttgccttttcagattatagaagtaatatgtgttcccatatttggcgtctctcaggagctcaggaagtacttggctgagtgaacatgtccattgtggaaaaatggcaacaatatggattccatgggtatattttatagaagaatatgaagaaaagcagctacccctaaacccattgcacaagctgttcatgttaattctgtacccgacgctttccccacggggcctcccctcactctgaaatggcatccaggtccatcttgccctccacctctgcatggctctccatgccccatcgcctctcccagatcctagcactgggtccacactctcgccctgtccatttaggttgatgaaagcaggcagtcacccgggtgggccagtcttgcctgtgggaggaacatgcagtctcctgtctcatggtttgaagtgtgccaggaagcctggcccagcccacctccccctggagtccttcccaggaggaataaccccttaggtcattgactataagatgagttcgctcactggatccttcctctctgatgagacaggaagaaggtacacagtgaccaggtaggaggaggagagggagtagaaaggagggatgcgggtggctggtccctgcatttgcctgcttccctgcacgggtgtcccactggccgcctctgctcaccagtgtcatgggattctctcagaagatgaaaacagcccctgcttttttgctagaatggctgagctttcatggaaaggaagctggacccaagcaacagccgactaccgaaggttgcctggagcagtgcagatgtgggaggaagaagggccttggtgcacactggcttttcttcctgactgcaatgtggcattgtgccagctacctcctctttctcggcctcaggaaaatggagagaaagcagccctgaaggtggctgtgacgagggaaggggcagagggcctgacagtcaaccacgcgctatattttcctgttcttccttagggcaagaactgcatggccagactcaggcaaggcctaggtgtgggctgggcattgcctacacgtgaagagatcactccgcgtccctactgcacctgtcacaaagtgccttctgatatgcctggcaaaccaaaatcggtgagcgccagcttgcttccctagaagacatttctaaatattcataacatgcttgctcaaatcaatcaccttattttacatccgctccagggagaaatgaagacatggtcctacgttgttctgtaattattttctatgtaaattttgttccttgttacaattatatatgtcttaggggaaaggaccatttcacatgtgtcacctcatgtgattctcaccacagccctgtgattgctcctgttttataaataatgacatagttccagttgatggccaaagccacagctaacgagaggcagagagagctcaggctcccaggagcttccactctcagaccttgcctcccgggctgccctgagtgaaacgcctgcttagcatttggcacagccagaagcagcaagctagggtcacaacacagagaggggctgtgtaatactggctgcctctgtgctaagaaaaaaaaaaaatcactgtgtgtttgtttattttggtgcaggcccagtgttcttgcttagacttaatactacccttcatgttaaaataaaaccaaacaaaaaccca

SEQ ID NO: 59 - RNA, 936 nt, synthetic construct
  source 1..936: mol_type = other RNA
atctccctccagcatttgtttctggaaggagtcaacaccaacagctctgacctgggcagccttcctgagaaaatgcagccattcctcctcctgttggcctttcttctgacccctggggctgggacagaggagatcatcgggggccatgaggccaagccccactcccgcccctacatggcctttgttcagtttctgcaagagaagagtcggaagaggtgtggcggcatcctagtgagaaaggactttgtgctgacagctgctcactgccagggaagctccataaatgtcaccttgggggcccacaatatcaaggaacaggagcggacccagcagtttatccctgtgaaaagacccatcccccatccagcctataatcctaagaacttctccaacgacatcatgctactgcagctggagagaaaggccaagtggaccacagctgtgcggcctctcaggctacctagcagcaaggcccaggtgaagccagggcagctgtgcagtgtggctggctggggttatgtctcaatgagcactttagcaaccacactgcaggaagtgttgctgacagtgcagaaggactgccagtgtgaacgtctcttccatggcaattacagcagagccactgagatttgtgtgggggatccaaagaagacacagaccggtttcaagggggactccggggggcccctcgtgtgtaaggacgtagcccaaggtattctctcctatggaaacaaaaaagggacacctccaggagtctacatcaaggtctcacacttcctgccctggataaagagaacaatgaagcgcctctaacagcaggcatgagactaaccttcctctgggcctgaccatctctgggacagaggcaagaatccccaaggggtgggcagtcggggttgcaggactgtaataaatggatctctggtgtaaatatga

SEQ ID NO: 60 - RNA, 5700 nt, synthetic construct
  source 1..5700: mol_type = other RNA
agcagccagcagtgactgcccgccctatctgggacccaggatcgctctgtgagcaacttggagccagagaggagatcaacaaggaggaggagagagccggcccctcagccctgctgcccagcagcagcctgtgctcgccctgcccaacgcagacagccagacccagggcggcccctctggcggctctgctcctcccgaaggatgcttggggagtgaggcgaagctgggccgctcctctcccctacagcagcccccttcctccatccctctgttctcctgagccttcaggagcctgcaccagtcctgcctgtccttctactcagctgttacccactctgggaccagcagtctttctgataactgggagagggcagtaaggaggacttcctggagggggtgactgtccagagcctggaactgtgcccacaccagaagccatcagcagcaaggacaccatgcggcttccgggtgcgatgccagctctggccctcaaaggcgagctgctgttgctgtctctcctgttacttctggaaccacagatctctcagggcctggtcgtcacacccccggggccagagcttgtcctcaatgtctccagcaccttcgttctgacctgctcgggttcagctccggtggtgtgggaacggatgtcccaggagcccccacaggaaatggccaaggcccaggatggcaccttctccagcgtgctcacactgaccaacctcactgggctagacacgggagaatacttttgcacccacaatgactcccgtggactggagaccgatgagcggaaacggctctacatctttgtgccagatcccaccgtgggcttcctccctaatgatgccgaggaactattcatctttctcacggaaataactgagatcaccattccatgccgagtaacagacccacagctggtggtgacactgcacgagaagaaaggggacgttgcactgcctgtcccctatgatcaccaacgtggcttttctggtatctttgaggacagaagctacatctgcaaaaccaccattggggacagggaggtggattctgatgcctactatgtctacagactccaggtgtcatccatcaacgtctctgtgaacgcagtgcagactgtggtccgccagggtgagaacatcaccctcatgtgcattgtgatcgggaatgaggtggtcaacttcgagtggacatacccccgcaaagaaagtgggcggctggtggagccggtgactgacttcctcttggatatgccttaccacatccgctccatcctgcacatccccagtgccgagttagaagactcggggacctacacctgcaatgtgacggagagtgtgaatgaccatcaggatgaaaaggccatcaacatcaccgtggttgagagcggctacgtgcggctcctgggagaggtgggcacactacaatttgctgagctgcatcggagccggacactgcaggtagtgttcgaggcctacccaccgcccactgtcctgtggttcaaagacaaccgcaccctgggcgactccagcgctggcgaaatcgccctgtccacgcgcaacgtgtcggagacccggtatgtgtcagagctgacactggttcgcgtgaaggtggcagaggctggccactacaccatgcgggccttccatgaggatgctgaggtccagctctccttccagctacagatcaatgtccctgtccgagtgctggagctaagtgagagccaccctgacagtggggaacagacagtccgctgtcgtggccggggcatgccccagccgaacatcatctggtctgcctgcagagacctcaaaaggtgtccacgtgagctgccgcccacgctgctggggaacagttccgaagaggagagccagctggagactaacgtgacgtactgggaggaggagcaggagtttgaggtggtgagcacactgcgtctgcagcacgtggatcggccactgtcggtgcgctgcacgctgcgcaacgctgtgggccaggacacgcaggaggtcatcgtggtgccacactccttgccctttaaggtggtggtgatctcagccatcctggccctggtggtgctcaccatcatctcccttatcatcctcatcatgctttggcagaagaagccacgttacgagatccgatggaaggtgattgagtctgtgagctctgacggccatgagtacatctacgtggaccccatgcagctgccctatgactccacgtgggagctgccgcgggaccagcttgtgctgggacgcaccctcggctctggggcctttgggcaggtggtggaggccacggctcatggcctgagccattctcaggccacgatgaaagtggccgtcaagatgcttaaatccacagcccgcagcagtgagaagcaagcccttatgtcggagctgaagatcatgagtcaccttgggccccacctgaacgtggtcaacctgttgggggcctgcaccaaaggaggacccatctatatcatcactgagtactgccgctacggagacctggtggactacctgcaccgcaacaaacacaccttcctgcagcaccactccgacaagcgccgcccgcccagcgcggagctctacagcaatgctctgcccgttgggctccccctgcccagccatgtgtccttgaccggggagagcgacggtggctacatggacatgagcaaggacgagtcggtggactatgtgcccatgctggacatgaaaggagacgtcaaatatgcagacatcgagtcctccaactacatggccccttacgataactacgttccctctgcccctgagaggacctgccgagcaactttgatcaacgagtctccagtgctaagctacatggacctcgtgggcttcagctaccaggtggccaatggcatggagtttctggcctccaagaactgcgtccacagagacctggcggctaggaacgtgctcatctgtgaaggcaagctggtcaagatctgtgactttggcctggctcgagacatcatgcgggactcgaattacatctccaaaggcagcacctttttgcctttaaagtggatggctccggagagcatcttcaacagcctctacaccaccctgagcgacgtgtggtccttcgggatcctgctctgggagatcttcaccttgggtggcaccccttacccagagctgcccatgaacgagcagttctacaatgccatcaaacggggttaccgcatggcccagcctgcccatgcctccgacgagatctatgagatcatgcagaagtgctgggaagagaagtttgagattcggccccccttctcccagctggtgctgcttctcgagagactgttgggcgaaggttacaaaaagaagtaccagcaggtggatgaggagtttctgaggagtgaccacccagccatccttcggtcccaggcccgcttgcctgggttccatggcctccgatctcccctggacaccagctccgtcctctatactgccgtgcagcccaatgagggtgacaacgactatatcatccccctgcctgaccccaaacccgaggttgctgacgagggcccactggagggttcccccagcctagccagctccaccctgaatgaagtcaacacctcctcaaccatctcctgtgacagccccctggagccccaggacgaaccagagccagagccccagcttgagctccaggtggagccggagccagagctggaacagttgccggattcggggtgccctgcgcctcgggcggaagcagaggatagcttcctgtagggggctggcccctaccctgccctgcctgaagctccccccctgccagcacccagcatctcctggcctggcctgaccgggcttcctgtcagccaggctgcccttatcagctgtccccttctggaagctttctgctcctgacgtgttgtgccccaaaccctggggctggcttaggaggcaagaaaactgcaggggccgtgaccagccctctgcctccagggaggccaactgactctgagccagggttcccccagggaactcagttttcccatatgtaaaatgggaaagttaggcttgatgacccagaatctaggattctctccctggctgacaggtggggagaccgaatccctccctgggaagattcttggagttactgaggtggtaaattaacttttttctgttcagccagctacccctcaaggaatcatagctctctcctcgcacttttatccacccaggagctagggaagagaccctagcctccctggctgctggctgagctagggcctagccttgagcagtgttgcctcatccagaagaaagccagtctcctccctatgatgccagtccctgcgttccctggcccgagctggtctggggccattaggcagcctaattaatgctggaggctgagccaagtacaggacacccccagcctgcagcccttgcccagggcacttggagcacacgcagccatagcaagtgcctgtgtccctgtccttcaggcccatcagtcctggggctttttctttatcaccctcagtcttaatccatccaccagagtctagaaggccagacgggccccgcatctgtgatgagaatgtaaatgtgccagtgtggagtggccacgtgtgtgtgccagtatatggccctggctctgcattggacctgctatgaggctttggaggaatccctcaccctctctgggcctcagtttccccttcaaaaaatgaataagtcggacttattaactctgagtgccttgccagcactaacattctagagtattccaggtggttgcacatttgtccagatgaagcaaggccatataccctaaacttccatcctgggggtcagctgggctcctgggagattccagatcacacatcacactctggggactcaggaaccatgccccttccccaggcccccagcaagtctcaagaacacagctgcacaggccttgacttagagtgacagccggtgtcctggaaagcccccagcagctgccccagggacatgggaagaccacgggacctctttcactacccacgatgacctccgggggtatcctgggcaaaagggacaaagagggcaaatgagatcacctcctgcagcccaccactccagcacctgtgccgaggtctgcgtcgaagacagaatggacagtgaggacagttatgtcttgtaaaagacaagaagcttcagatgggtaccccaagaaggatgtgagaggtgggcgctttggaggtttgcccctcacccaccagctgccccatccctgaggcagcgctccatgggggtatggttttgtcactgcccagacctagcagtgacatctcattgtccccagcccagtgggcattggaggtgccaggggagtcagggttgtagccaagacgcccccgcacggggagggttgggaagggggtgcaggaagctcaacccctctgggcaccaaccctgcattgcaggttggcaccttacttccctgggatccccagagttggtccaaggagggagagtgggttctcaatacggtaccaaagatataatcacctaggtttacaaatatttttaggactcacgttaactcacatttatacagcagaaatgctattttgtatgctgttgagtttttctatctgtgtacttttttttaagggaaagattttaatattaaacctggtgcttctcactcaca